European Patent Specification EP 3 889 166 B1, published August 6, 2025. Title: PRRSV minor protein-containing recombinant viral vectors and methods of making and use thereof. Applicant: Boehringer Ingelheim Animal Health USA Inc. Application PCT/US2016/038964. The sequence listing filed with the application follows.

SEQUENCE LISTING (139 sequences)

SEQ ID NO: 1 - protein, 256 aa, Artificial Sequence
  PRRS gp2
MKWGPCKAFLTKLANFLWMLSRSSWCPLLISLYFWPFCLASPSPVGWWSFASDWFAPRYSVRALPFTLSNYRRSYEAFLSQCQVDIPTWGTKHPLGMLWHHKVSTLIDEMVSRRMYRIMEKAGQAAWKQVVSEATLSRISSLDVVAHFQHLAAIEAETCKYLASRLPMLHNLRMTGSNVTIVYNSTLNQVFAIFPTPGSRPKLHDFQQWLIAVHSSIFSSVAASCTLFVVLWLRVPILRTVFGFRWLGAIFLSNSQ

SEQ ID NO: 2 - DNA, 768 bp, Artificial Sequence
  VR2332 PRRSV gp2
atgaaatggggtccatgcaaagcctttttgacaaaattggccaactttttgtggatgctttcacggagttcttggtgtccattgttgatatcattatatttttggccattttgtttggcttcaccatcgccggttggctggtggtcttttgcatcagattggtttgctccgcgatactccgtacgcgccctgccattcactctgagcaattacagaagatcttatgaggcctttctttcccagtgccaagtggacattcccacctggggaactaaacatcctttggggatgctttggcaccataaggtgtcaaccctgattgatgaaatggtgtcgcgtcgaatgtaccgcatcatggaaaaagcagggcaggctgcctggaaacaggtggtgagcgaggctacgctgtctcgcattagtagtttggatgtggtggctcattttcagcatctagccgccattgaagccgagacctgtaaatatttggcctcccggctgcccatgctacacaacctgcgcatgacagggtcaaatgtaaccatagtgtataatagcactttgaatcaggtgtttgctatttttccaacccctggttcccggccaaagcttcatgattttcagcaatggttaatagctgtacattcctccatattttcctctgttgcagcttcttgtactctttttgttgtgctgtggttgcgggttccaatactacgtactgtttttggtttccgctggttaggggcaatttttctttcgaactcacag

SEQ ID NO: 3 - protein, 254 aa, Artificial Sequence
  PRRSV gp3
MVNSCTFLHIFLCCSFLYSFCCAVVAGSNTTYCFWFPLVRGNFSFELTVNYTVCPPCLTRQAATEIYEPGRSLWCRIGYDRCGEDDHDELGFMIPPGLSSEGHLTGVYAWLAFLSFSYTAQFHPEIFGIGNVSRVYVDIKHQLICAEHDGQNTTLPRHDNISAVFQTYYQHQVDGGNWFHLEWLRPFFSSWLVLNVSWFLRRSPANHVSVRVLQILRPTPPQRQALLSSKTSVALGIATRPLRRFAKSLSAVRR

SEQ ID NO: 4 - DNA, 762 bp, Artificial Sequence
  VR2332 PRRSV gp3 (12696..13460 of VR2332)
atggttaatagctgtacattcctccatattttcctctgttgcagcttcttgtactctttttgttgtgctgtggttgcgggttccaatactacgtactgtttttggtttccgctggttaggggcaatttttctttcgaactcacagtgaattacacggtgtgtccaccttgcctcacccggcaagcagccacagagatctacgaacccggtaggtctctttggtgcaggatagggtatgaccgatgtggggaggacgatcatgacgagctagggtttatgataccgcctggcctctccagcgaaggccacttgactggtgtttacgcctggttggcgttcttgtccttcagctacacggcccagttccatcccgagatattcgggatagggaatgtgagtcgagtttatgttgacatcaaacatcaactcatctgcgccgaacatgacgggcagaacaccaccttgcctcgtcatgacaacatttcagccgtgtttcagacctattaccaacatcaagtcgacggcggcaattggtttcacctagaatggcttcgtcccttcttttcctcgtggttggttttaaatgtctcttggtttctcaggcgttcgcctgcaaaccatgtttcagttcgagtcttgcagatattaagaccaacaccaccgcagcggcaagctttgctgtcctccaagacatcagttgccttaggcatcgcgactcggcctctgaggcgattcgcaaaatccctcagtgccgtacggcga

SEQ ID NO: 5 - protein, 178 aa, Artificial Sequence
  PRRSV gp4 polypeptide (VR2332)
MASSLLFLVVGFKCLLVSQAFACKPCFSSSLADIKTNTTAAASFAVLQDISCLRHRDSASEAIRKIPQCRTAIGTPVYVTITANVTDENYLHSSDLLMLSSCLFYASEMSEKGFKVVFGNVSGIVAVCVNFTSYVQHVKEFTQRSLVVDHVRLLHFMTPETMRWATVLACLFAILLAI

SEQ ID NO: 6 - DNA, 534 bp, Artificial Sequence
  VR2332 PRRSV gp4 (13241..13777 of VR2332)
atggcttcgtcccttcttttcctcgtggttggttttaaatgtctcttggtttctcaggcgttcgcctgcaaaccatgtttcagttcgagtcttgcagatattaagaccaacaccaccgcagcggcaagctttgctgtcctccaagacatcagttgccttaggcatcgcgactcggcctctgaggcgattcgcaaaatccctcagtgccgtacggcgatagggacacccgtgtatgttaccatcacagccaatgtgacagatgagaattatttacattcttctgatctcctcatgctttcttcttgccttttctatgcttctgagatgagtgaaaagggatttaaggtggtatttggcaatgtgtcaggcatcgtggctgtgtgtgtcaattttaccagctacgtccaacatgtcaaggagtttacccaacgctccctggtggtcgaccatgtgcggttgctccatttcatgacacctgagaccatgaggtgggcaactgttttagcctgtctttttgccattctgttggcaatt

SEQ ID NO: 7 - protein, 73 aa, Artificial Sequence
  PRRSV E polypeptide (VR2332)
MGSMQSLFDKIGQLFVDAFTEFLVSIVDIIIFLAILFGFTIAGWLVVFCIRLVCSAILRTRPAIHSEQLQKIL

SEQ ID NO: 8 - DNA, 219 bp, Artificial Sequence
  VR2332 PRRSV E (12078..12299 of VR2332)
atggggtccatgcaaagcctttttgacaaaattggccaactttttgtggatgctttcacggagttcttggtgtccattgttgatatcattatatttttggccattttgtttggcttcaccatcgccggttggctggtggtcttttgcatcagattggtttgctccgcgatactccgtacgcgccctgccattcactctgagcaattacagaagatctta

SEQ ID NO: 9 - DNA, 768 bp, Artificial Sequence
  VR2332 PRRSV gp2 (codon-optimized)
atgaaatggggaccctgtaaggctttcctgactaaactcgcaaacttcctctggatgctctcacgatcttcctggtgccctctgctcatctctctctacttctggccattttgcctggcctccccctctccagtgggatggtggtcattcgccagtgactggtttgctccccgatattcagtgcgggctctcccattcactctgagcaactaccggcgctcctatgaggcatttctgagccagtgtcaggtggacatcccaacctggggcacaaagcaccctctgggaatgctctggcaccataaagtgagtacactgatcgatgagatggtcagcaggagaatgtacagaattatggaaaaggctggccaggccgcttggaaacaggtggtctctgaagcaaccctctcacgaatcagctccctggacgtggtcgcccacttccagcatctcgcagccattgaggcagaaacatgcaagtacctggccagccgcctgcctatgctccataacctgaggatgactgggtccaatgtgaccatcgtctataactctacactgaatcaggtgttcgctatttttcctactcccggcagcaggcccaaactccacgatttccagcagtggctgatcgccgtgcattcttcaattttcagtagcgtcgctgcatcctgtaccctgtttgtggtcctgtggctccgggtgcccatcctccgcacagtgttcgggtttcggtggctgggggctattttcctctccaactcacag

SEQ ID NO: 10 - DNA, 762 bp, Artificial Sequence
  VR2332 PRRSV gp3 (codon-optimized)
atggtcaattcctgtaccttcctccacatcttcctctgttgttcattcctctattccttctgttgcgctgtcgtcgctgggtcaaacaccacatactgcttctggtttccactggtgagaggaaacttctcctttgagctcacagtcaattataccgtgtgccctccatgtctgacccgacaggcagctacagaaatctacgaacctggcaggtctctgtggtgcagaattggctatgaccgatgtggagaggacgatcacgatgaactggggttcatgatccctcccggcctgagctccgaaggacatctcacaggggtctacgcatggctggccttcctctccttttcttatactgcccagttccaccccgaaatcttcgggattggcaacgtgtccagggtgtacgtcgacatcaagcaccagctgatttgtgccgaacatgacggccagaacactaccctgcctcggcatgataatatcagcgccgtgttccagacctactatcagcaccaggtggatggcggaaattggtttcatctggagtggctccggcccttcttttcttcatggctggtcctcaacgtgtcatggttcctgcggcgcagtcccgccaatcacgtgagcgtccgggtgctgcagattctccgcccaactccacctcagaggcaggctctgctcagtagcaaaacctcagtggcactgggcatcgctacacgacctctcagacggttcgctaagtccctctcagcagtcagaagg

SEQ ID NO: 11 - DNA, 534 bp, Artificial Sequence
  VR2332 PRRSV gp4 (codon-optimized)
atggcttcatctctcctcttcctcgtcgtgggattcaaatgtctgctcgtgtctcaggccttcgcttgtaaaccctgcttttccagtagcctggctgacatcaagactaacaccacagccgctgcatcattcgcagtgctgcaggacattagttgcctccgacaccgagatagtgccagcgaggctatcaggaaaattccccagtgtagaacagcaatcgggactccagtgtacgtcactattaccgccaacgtgacagacgaaaattatctgcatagctccgatctgctcatgctgtcttcatgcctcttctacgcttccgagatgtctgaaaagggcttcaaagtggtctttggcaacgtctctggaatcgtggccgtgtgcgtgaatttcaccagctatgtccagcacgtgaaggagtttacacagcgatccctggtggtcgatcacgtgcgcctgctccacttcatgacccctgaaaccatgcggtgggctactgtcctcgcctgcctgttcgccattctcctcgctatt

SEQ ID NO: 12 - DNA, 219 bp, Artificial Sequence
  VR2332 PRRSV E (codon-optimized)
atggggtctatgcagtcactgtttgataagattgggcagctctttgtggacgcctttaccgagttcctggtcagcattgtggacatcatcattttcctggccatcctcttcggctttaccattgctggatggctggtggtcttttgcatccggctcgtgtgtagcgccatcctcagaacaagacctgccatccactccgaacagctccagaaaatcctc

SEQ ID NO: 13 - DNA, 816 bp, Artificial Sequence
  VR2332 PRRSV rtg-gp2 DNA (codon-optimized, re-targeted)
atggatgctatgaaacggggactctgttgcgtgctgctgctgtgcggagccgtctttgtctcaccttcctcaccaagccctgtcgggtggtggtcctttgcttctgactggttcgcaccacgatactccgtgcgggcactgccttttactctctccaactaccggcgctcttatgaggccttcctgtctcagtgccaggtggacatccctacctggggaacaaagcaccccctcgggatgctgtggcaccataaagtgtctacactgatcgatgagatggtctcaaggagaatgtatagaattatggaaaaggcaggccaggccgcttggaaacaggtggtctcagaagccaccctgagtcgaatcagctccctcgatgtggtcgctcactttcagcatctggcagccattgaggccgaaacctgtaagtacctcgctagccgcctccccatgctgcacaacctcaggatgactggcagtaatgtgaccatcgtctataacagcacactgaatcaggtgtttgctattttccccactccaggaagcaggccaaagctgcatgacttccagggcggaagcgagcagaaactgatctccgaggaggacctgggaggatcaggaggaagtggaggatccgagctggtggaagggtggttttcttcatggaagagtagcatcgcctccttctttttcatcattgggctgatcattggcctgttcctcgtgctgcgggtcggaatccatctgtgcatcaagctgaaacatacaaagaaacgacagatttacactgacattgagatgaatagactgggcaaa

SEQ ID NO: 14 - protein, 272 aa, Artificial Sequence
  VR2332 PRRSV rtg-gp2 polypeptide (gp2-myc-VSV)
MDAMKRGLCCVLLLCGAVFVSPSSPSPVGWWSFASDWFAPRYSVRALPFTLSNYRRSYEAFLSQCQVDIPTWGTKHPLGMLWHHKVSTLIDEMVSRRMYRIMEKAGQAAWKQVVSEATLSRISSLDVVAHFQHLAAIEAETCKYLASRLPMLHNLRMTGSNVTIVYNSTLNQVFAIFPTPGSRPKLHDFQGGSEQKLISEEDLGGSGGSGGSELVEGWFSSWKSSIASFFFIIGLIIGLFLVLRVGIHLCIKLKHTKKRQIYTDIEMNRLGK

SEQ ID NO: 15 - DNA, 759 bp, Artificial Sequence
  VR2332 PRRSV rtg-gp3 DNA (codon-optimized, re-targeted)
atggatgctatgaaacgggggctctgctgcgtcctcctcctgtgcggggctgtcttcgtctcaccctcctcaaatacaacctactgcttttggttcccactcgtgagaggcaactttagcttcgagctgactgtgaattacaccgtctgccctccatgtctgacccgacaggccgctgcagaaatctacgaacctggacggtccctgtggtgccgcattgggtatgacaggtgtgaggaagacgatcacgatgagctgggctttatggtgcctcctggactcagctccgaaggacatctgacatcagtctacgcctggctcgcttttctgtccttctcttatactgctcagtttcaccccgaaatcttcggaattgggaacgtgtctcgggtgtacgtcgacatcaagcaccagctcatttgcgcagaacatgacggccagaacaccacactgccaaggcacgataatatctccgccgtgttccagacatactatcagcatcaggtcgacggcggagggggctctgattataaggacgatgacgataaaggagggtcaggcggaagtgggggatccgagctggtggaaggctggttttcttcatggaagagtagcatcgccagcttctttttcatcattggcctcatcattggactgttcctcgtgctgcgcgtcggaatccacctgtgcatcaagctgaagcatactaagaagcggcagatttacaccgacattgagatgaacagactggggaaatga

SEQ ID NO: 16 - protein, 252 aa, Artificial Sequence
  VR2332 PRRSV rtg-gp3 polypeptide (gp3-Flag-VSV)
MDAMKRGLCCVLLLCGAVFVSPSSNTTYCFWFPLVRGNFSFELTVNYTVCPPCLTRQAAAEIYEPGRSLWCRIGYDRCEEDDHDELGFMVPPGLSSEGHLTSVYAWLAFLSFSYTAQFHPEIFGIGNVSRVYVDIKHQLICAEHDGQNTTLPRHDNISAVFQTYYQHQVDGGGGSDYKDDDDKGGSGGSGGSELVEGWFSSWKSSIASFFFIIGLIIGLFLVLRVGIHLCIKLKHTKKRQIYTDIEMNRLGK

SEQ ID NO: 17 - DNA, 714 bp, Artificial Sequence
  VR2332 PRRSV rtg-gp4 DNA (codon-optimized, re-targeted)
atggatgctatgaaacggggactgtgctgcgtgctgctgctctgtggggctgtcttcgtgtcaccttcttgtaaaccttgcttttccagctccctggctgacatcaagactaacaccacagccgctgcatcttttgcagtgctccaggacatttcatgcctgcgacaccgagatagcgcctccgaggctatcaggaaaattcctcagtgtagaacagcaatcggcactcccgtgtacgtcactattaccgccaacgtgacagacgaaaattatctgcattctagcgacctgctcatgctcagtagctgcctgttctacgcctctgagatgtcagaaaagggctttaaagtggtcttcgggaacgtgagcggcatcgtggccgtgtgcgtgaacttcaccagctatgtccagcacgtgaaggagttcacacagcgatccctggtggtcgatcacgtccgcctgctccatggcggatcttacccctatgacgtgccagattacgcaggaggaagtggaggaagcggaggatccgagctggtggaaggatggttttcctcttggaagtcaagtatcgccagcttctttttcatcattggactcatcattgggctgttcctcgtcctgcgggtgggaatccatctgtgcatcaagctgaagcatacaaagaagcggcagatttacactgacattgagatgaatagactgggcaaatga

SEQ ID NO: 18 - protein, 237 aa, Artificial Sequence
  VR2332 PRRSV rtg-gp4 polypeptide (gp4-HA-VSV)
MDAMKRGLCCVLLLCGAVFVSPSCKPCFSSSLADIKTNTTAAASFAVLQDISCLRHRDSASEAIRKIPQCRTAIGTPVYVTITANVTDENYLHSSDLLMLSSCLFYASEMSEKGFKVVFGNVSGIVAVCVNFTSYVQHVKEFTQRSLVVDHVRLLHGGSYPYDVPDYAGGSGGSGGSELVEGWFSSWKSSIASFFFIIGLIIGLFLVLRVGIHLCIKLKHTKKRQIYTDIEMNRLGK

SEQ ID NO: 19 - DNA, 10 bp, Artificial Sequence
  Place holder for: VR2332 PRRSV rtg-E (codon-optimized, re-targeted)
  misc_feature (1)..(10): n is a, c, g, t or u
nnnnnnnnnn

SEQ ID NO: 20 - protein, 10 aa, Artificial Sequence
  Placeholder for: VR2332 PRRSV rtg-E polypeptide
  misc_feature (1)..(10): Xaa can be any naturally occurring amino acid
XXXXXXXXXX

SEQ ID NO: 21 - DNA, 4566 bp, Artificial Sequence
  vAD3038 insert cassette
aaataatgattttattttgactgatagtgacctgttcgttgcaacacattgatgagcaatgcttttttataatgccaactttgtacaaaaaagcaggtcgactctagaggatccgaaaaaacctcccacacctccccctgaacctgaaacataaaatgaatgcaattgttgttgttaacttgtttattgcagcttataatggttacaaataaagcaatagcatcacaaatttcacaaataaagcatttttttcactgcattctagttgtggtttgtccaaactcatcaatgtatcttatcatgtctggatccccaagcttctcgagaccggttcatttgcccagtctattcatctcaatgtcagtgtaaatctgtcgtttctttgtatgtttcagcttgatgcacagatggattccgacccgcagcacgaggaacaggccaatgatcagcccaatgatgaaaaagaaggaggcgatgctactcttccatgaagaaaaccacccttccaccagctcggatcctccacttcctcctgatcctcccaggtcctcctcggagatcagtttctgctcgcttccgccctggaagtcatgcagctttggcctgcttcctggagtggggaaaatagcaaacacctgattcagtgtgctgttatagacgatggtcacattactgccagtcatcctgaggttgtgcagcatggggaggcggctagcgaggtacttacaggtttcggcctcaatggctgccagatgctgaaagtgagcgaccacatcgagggagctgattcgactcagggtggcttctgagaccacctgtttccaagcggcctggcctgccttttccataattctatacattctccttgagaccatctcatcgatcagtgtagacactttatggtgccacagcatcccgagggggtgctttgttccccaggtagggatgtccacctggcactgagacaggaaggcctcataagagcgccggtagttggagagagtaaaaggcagtgcccgcacggagtatcgtggtgcgaaccagtcagaagcaaaggaccaccacccgacagggcttggtgaggaaggtgagacaaagacggctccgcacagcagcagcacgcaacagagtccccgtttcatagcatccatggtttaattaaagctttttgcaaaagcctaggcctccaaaaaagcctcctcactacttctggaatagctcagaggccgaggcggcctcggcctctgcataaataaaaaaaattagtcagccatggggcggagaatgggcggaactgggcggagttaggggcgggatgggcggagttaggggcgggactatggttgctgactaattgagatgcatgctttgcatacttctgcctgctggggagcctggggactttccacacctggttgctgactaattgagatgcatgctttgcatacttctgcctgctggggagcctggggactttccacaccctaactgacacacattccacagccaagctgtaccgagctcgaattcgctagcatcgatgcggccgcgttgacattgattattgactagttattaatagtaatcaattacggggtcattagttcatagcccatatatggagttccgcgttacataacttacggtaaatggcccgcctggctgaccgcccaacgacccccgcccattgacgtcaataatgacgtatgttcccatagtaacgccaatagggactttccattgacgtcaatgggtggactatttacggtaaactgcccacttggcagtacatcaagtgtatcatatgccaagtacgccccctattgacgtcaatgacggtaaatggcccgcctggcattatgcccagtacatgaccttatgggactttcctacttggcagtacatctacgtattagtcatcgctattaccatggtgatgcggttttggcagtacatcaatgggcgtggatagcggtttgactcacggggatttccaagtctccaccccattgacgtcaatgggagtttgttttggcaccaaaatcaacgggactttccaaaatgtcgtaacaactccgccccattgacgcaaatgggcggtaggcgtgtacggtgggaggtctatataagcagagctctctagaaccatggatgctatgaaacggggactgtgctgcgtgctgctgctctgtggggctgtcttcgtgtcaccttcttgtaaaccttgcttttccagctccctggctgacatcaagactaacaccacagccgctgcatcttttgcagtgctccaggacatttcatgcctgcgacaccgagatagcgcctccgaggctatcaggaaaattcctcagtgtagaacagcaatcggcactcccgtgtacgtcactattaccgccaacgtgacagacgaaaattatctgcattctagcgacctgctcatgctcagtagctgcctgttctacgcctctgagatgtcagaaaagggctttaaagtggtcttcgggaacgtgagcggcatcgtggccgtgtgcgtgaacttcaccagctatgtccagcacgtgaaggagttcacacagcgatccctggtggtcgatcacgtccgcctgctccatggcggatcttacccctatgacgtgccagattacgcaggaggaagtggaggaagcggaggatccgagctggtggaaggatggttttcctcttggaagtcaagtatcgccagcttctttttcatcattggactcatcattgggctgttcctcgtcctgcgggtgggaatccatctgtgcatcaagctgaagcatacaaagaagcggcagatttacactgacattgagatgaatagactgggcaaatgatgacccccccccctaacgttactggccgaagccgcttggaataaggccggtgtgcgtttgtctatatgttattttccaccatattgccgtcttttggcaatgtgagggcccggaaacctggccctgtcttcttgacgagcattcctaggggtctttcccctctcgccaaaggaatgcaaggtctgttgaatgtcgtgaaggaagcagttcctctggaagcttcttgaagacaaacaacgtctgtagcgaccctttgcaggcagcggaaccccccacctggcgacaggtgcctctgcggccaaaagccacgtgtataagatacacctgcaaaggcggcacaaccccagtgccacgttgtgagttggatagttgtggaaagagtcaaatggctctcctcaagcgtattcaacaaggggctgaaggatgcccagaaggtaccccattgtatgggatctgatctggggcctcggtgcacatgctttacatgtgtttagtcgaggttaaaaaacgtctaggccccccgaaccacggggacgtggttttcctttgaaaaacacgatgataataccatggatgctatgaaacgggggctctgctgcgtcctcctcctgtgcggggctgtcttcgtctcaccctcctcaaatacaacctactgcttttggttcccactcgtgagaggcaactttagcttcgagctgactgtgaattacaccgtctgccctccatgtctgacccgacaggccgctgcagaaatctacgaacctggacggtccctgtggtgccgcattgggtatgacaggtgtgaggaagacgatcacgatgagctgggctttatggtgcctcctggactcagctccgaaggacatctgacatcagtctacgcctggctcgcttttctgtccttctcttatactgctcagtttcaccccgaaatcttcggaattgggaacgtgtctcgggtgtacgtcgacatcaagcaccagctcatttgcgcagaacatgacggccagaacaccacactgccaaggcacgataatatctccgccgtgttccagacatactatcagcatcaggtcgacggcggagggggctctgattataaggacgatgacgataaaggagggtcaggcggaagtgggggatccgagctggtggaaggctggttttcttcatggaagagtagcatcgccagcttctttttcatcattggcctcatcattggactgttcctcgtgctgcgcgtcggaatccacctgtgcatcaagctgaagcatactaagaagcggcagatttacaccgacattgagatgaacagactggggaaatgatgaggtaccgggggaggctaactgaaacacggaaggagacaataccggaaggaacccgcgctatgacggcaataaaaagacagaataaaacgcacgggtgttgggtcgtttgttcataaacgcggggttcggtcccagggctggcactctgtcgataccccaccgagaccccattggggccaatacgcccgcgtttcttccttttccccaccccaccccccaagttcgggtgaaggcccagggctcgcagccaacgtcggggcggcaggccctgccatagccagctttcttgtacaaagttggcattataagaaagcattgcttatcaatttgttgcaacgaacaggtcactatcagtcaaaataaaatcattattt

SEQ ID NO: 22 - DNA, 4662 bp, Artificial Sequence
  pAD3041 transgene cassette
aaataatgattttattttgactgatagtgacctgttcgttgcaacacattgatgagcaatgcttttttataatgccaactttgtacaaaaaagcaggtcgactctagaggatccgaaaaaacctcccacacctccccctgaacctgaaacataaaatgaatgcaattgttgttgttaacttgtttattgcagcttataatggttacaaataaagcaatagcatcacaaatttcacaaataaagcatttttttcactgcattctagttgtggtttgtccaaactcatcaatgtatcttatcatgtctggatccccaagcttctcgagaccggtcctgcaggtcagaggattttctggagctgttcggagtggatggcaggtcttgttctgaggatggcgctacacacgagccggatgcaaaagaccaccagccatccagcaatggtaaagccgaagaggatggccaggaaaatgatgatgtccacaatgctgaccaggaactcggtaaaggcgtccacaaagagctgcccaatcttatcaaacagtgactgcatagaccccatggtggaggtccagggttctcctccacgtctccagcctgcttcagcaggctgaagttagtagctccgcttcccctgcaggtcactgtgagttggagaggaaaatagcccccagccaccgaaacccgaacactgtgcggaggatgggcacccggagccacaggaccacaaacagggtacaggatgcagcgacgctactgaaaattgaagaatgcacggcgatcagccactgctggaaatcgtggagtttgggcctgctgccgggagtaggaaaaatagcgaacacctgattcagtgtagagttatagacgatggtcacattggacccagtcatcctcaggttatggagcataggcaggcggctggccaggtacttgcatgtttctgcctcaatggctgcgagatgctggaagtgggcgaccacgtccagggagctgattcgtgagagggttgcttcagagaccacctgtttccaagcggcctggccagccttttccataattctgtacattctcctgctgaccatctcatcgatcagtgtactcactttatggtgccagagcattcccagagggtgctttgtgccccaggttgggatgtccacctgacactggctcagaaatgcctcataggagcgccggtagttgctcagagtgaatgggagagcccgcactgaatatcggggagcaaaccagtcactggcgaatgaccaccatcccactggagagggggaggccaggcaaaatggccagaagtagagagagatgagcagagggcaccaggaagatcgtgagagcatccagaggaagtttgcgagtttagtcaggaaagccttacagggtccccatttcatggtggagctttttgcaaaagcctaggcctccaaaaaagcctcctcactacttctggaatagctcagaggccgaggcggcctcggcctctgcataaataaaaaaaattagtcagccatggggcggagaatgggcggaactgggcggagttaggggcgggatgggcggagttaggggcgggactatggttgctgactaattgagatgcatgctttgcatacttctgcctgctggggagcctggggactttccacacctggttgctgactaattgagatgcatgctttgcatacttctgcctgctggggagcctggggactttccacaccctaactgacacacattccacagccaagctgtaccgagctcgaattcgctagcatcgatgcggccgcgttgacattgattattgactagttattaatagtaatcaattacggggtcattagttcatagcccatatatggagttccgcgttacataacttacggtaaatggcccgcctggctgaccgcccaacgacccccgcccattgacgtcaataatgacgtatgttcccatagtaacgccaatagggactttccattgacgtcaatgggtggactatttacggtaaactgcccacttggcagtacatcaagtgtatcatatgccaagtacgccccctattgacgtcaatgacggtaaatggcccgcctggcattatgcccagtacatgaccttatgggactttcctacttggcagtacatctacgtattagtcatcgctattaccatggtgatgcggttttggcagtacatcaatgggcgtggatagcggtttgactcacggggatttccaagtctccaccccattgacgtcaatgggagtttgttttggcaccaaaatcaacgggactttccaaaatgtcgtaacaactccgccccattgacgcaaatgggcggtaggcgtgtacggtgggaggtctatataagcagagctctctagaaccaccatggcttcatctctcctcttcctcgtcgtgggattcaaatgtctgctcgtgtctcaggccttcgcttgtaaaccctgcttttccagtagcctggctgacatcaagactaacaccacagccgctgcatcattcgcagtgctgcaggacattagttgcctccgacaccgagatagtgccagcgaggctatcaggaaaattccccagtgtagaacagcaatcgggactccagtgtacgtcactattaccgccaacgtgacagacgaaaattatctgcatagctccgatctgctcatgctgtcttcatgcctcttctacgcttccgagatgtctgaaaagggcttcaaagtggtctttggcaacgtctctggaatcgtggccgtgtgcgtgaatttcaccagctatgtccagcacgtgaaggagtttacacagcgatccctggtggtcgatcacgtgcgcctgctccacttcatgacccctgaaaccatgcggtgggctactgtcctcgcctgcctgttcgccattctcctcgctatttgaagatctcccccccccctaacgttactggccgaagccgcttggaataaggccggtgtgcgtttgtctatatgttattttccaccatattgccgtcttttggcaatgtgagggcccggaaacctggccctgtcttcttgacgagcattcctaggggtctttcccctctcgccaaaggaatgcaaggtctgttgaatgtcgtgaaggaagcagttcctctggaagcttcttgaagacaaacaacgtctgtagcgaccctttgcaggcagcggaaccccccacctggcgacaggtgcctctgcggccaaaagccacgtgtataagatacacctgcaaaggcggcacaaccccagtgccacgttgtgagttggatagttgtggaaagagtcaaatggctctcctcaagcgtattcaacaaggggctgaaggatgcccagaaggtaccccattgtatgggatctgatctggggcctcggtgcacatgctttacatgtgtttagtcgaggttaaaaaacgtctaggccccccgaaccacggggacgtggttttcctttgaaaaacacgatgataataccaccatggtcaattcctgtaccttcctccacatcttcctctgttgttcattcctctattccttctgttgcgctgtcgtcgctgggtcaaacaccacatactgcttctggtttccactggtgagaggaaacttctcctttgagctcacagtcaattataccgtgtgccctccatgtctgacccgacaggcagctacagaaatctacgaacctggcaggtctctgtggtgcagaattggctatgaccgatgtggagaggacgatcacgatgaactggggttcatgatccctcccggcctgagctccgaaggacatctcacaggggtctacgcatggctggccttcctctccttttcttatactgcccagttccaccccgaaatcttcgggattggcaacgtgtccagggtgtacgtcgacatcaagcaccagctgatttgtgccgaacatgacggccagaacactaccctgcctcggcatgataatatcagcgccgtgttccagacctactatcagcaccaggtggatggcggaaattggtttcatctggagtggctccggcccttcttttcttcatggctggtcctcaacgtgtcatggttcctgcggcgcagtcccgccaatcacgtgagcgtccgggtgctgcagattctccgcccaactccacctcagaggcaggctctgctcagtagcaaaacctcagtggcactgggcatcgctacacgacctctcagacggttcgctaagtccctctcagcagtcagaaggtgaagatctggtaccgggggaggctaactgaaacacggaaggagacaataccggaaggaacccgcgctatgacggcaataaaaagacagaataaaacgcacgggtgttgggtcgtttgttcataaacgcggggttcggtcccagggctggcactctgtcgataccccaccgagaccccattggggccaatacgcccgcgtttcttccttttccccaccccaccccccaagttcgggtgaaggcccagggctcgcagccaacgtcggggcggcaggccctgccatagccagctttcttgtacaaagttggcattataagaaagcattgcttatcaatttgttgcaacgaacaggtcactatcagtcaaaataaaatcattattt

SEQ ID NO: 23 - DNA, 4361 bp, Artificial Sequence
  vAD3042 transgene cassette
aaataatgattttattttgactgatagtgacctgttcgttgcaacacattgatgagcaatgcttttttataatgccaactttgtacaaaaaagcaggtcgactctagaggatccgaaaaaacctcccacacctccccctgaacctgaaacataaaatgaatgcaattgttgttgttaacttgtttattgcagcttataatggttacaaataaagcaatagcatcacaaatttcacaaataaagcatttttttcactgcattctagttgtggtttgtccaaactcatcaatgtatcttatcatgtctggatccccaagcttctcgagaccggtcctgcaggtcactgtgagttggagaggaaaatagcccccagccaccgaaacccgaacactgtgcggaggatgggcacccggagccacaggaccacaaacagggtacaggatgcagcgacgctactgaaaattgaagaatgcacggcgatcagccactgctggaaatcgtggagtttgggcctgctgccgggagtaggaaaaatagcgaacacctgattcagtgtagagttatagacgatggtcacattggacccagtcatcctcaggttatggagcataggcaggcggctggccaggtacttgcatgtttctgcctcaatggctgcgagatgctggaagtgggcgaccacgtccagggagctgattcgtgagagggttgcttcagagaccacctgtttccaagcggcctggccagccttttccataattctgtacattctcctgctgaccatctcatcgatcagtgtactcactttatggtgccagagcattcccagagggtgctttgtgccccaggttgggatgtccacctgacactggctcagaaatgcctcataggagcgccggtagttgctcagagtgaatgggagagcccgcactgaatatcggggagcaaaccagtcactggcgaatgaccaccatcccactggagagggggaggccaggcaaaatggccagaagtagagagagatgagcagagggcaccaggaagatcgtgagagcatccagaggaagtttgcgagtttagtcaggaaagccttacagggtccccatttcatggtggagctttttgcaaaagcctaggcctccaaaaaagcctcctcactacttctggaatagctcagaggccgaggcggcctcggcctctgcataaataaaaaaaattagtcagccatggggcggagaatgggcggaactgggcggagttaggggcgggatgggcggagttaggggcgggactatggttgctgactaattgagatgcatgctttgcatacttctgcctgctggggagcctggggactttccacacctggttgctgactaattgagatgcatgctttgcatacttctgcctgctggggagcctggggactttccacaccctaactgacacacattccacagccaagctgtaccgagctcgaattcgctagcatcgatgcggccgcgttgacattgattattgactagttattaatagtaatcaattacggggtcattagttcatagcccatatatggagttccgcgttacataacttacggtaaatggcccgcctggctgaccgcccaacgacccccgcccattgacgtcaataatgacgtatgttcccatagtaacgccaatagggactttccattgacgtcaatgggtggactatttacggtaaactgcccacttggcagtacatcaagtgtatcatatgccaagtacgccccctattgacgtcaatgacggtaaatggcccgcctggcattatgcccagtacatgaccttatgggactttcctacttggcagtacatctacgtattagtcatcgctattaccatggtgatgcggttttggcagtacatcaatgggcgtggatagcggtttgactcacggggatttccaagtctccaccccattgacgtcaatgggagtttgttttggcaccaaaatcaacgggactttccaaaatgtcgtaacaactccgccccattgacgcaaatgggcggtaggcgtgtacggtgggaggtctatataagcagagctctctagaaccaccatggcttcatctctcctcttcctcgtcgtgggattcaaatgtctgctcgtgtctcaggccttcgcttgtaaaccctgcttttccagtagcctggctgacatcaagactaacaccacagccgctgcatcattcgcagtgctgcaggacattagttgcctccgacaccgagatagtgccagcgaggctatcaggaaaattccccagtgtagaacagcaatcgggactccagtgtacgtcactattaccgccaacgtgacagacgaaaattatctgcatagctccgatctgctcatgctgtcttcatgcctcttctacgcttccgagatgtctgaaaagggcttcaaagtggtctttggcaacgtctctggaatcgtggccgtgtgcgtgaatttcaccagctatgtccagcacgtgaaggagtttacacagcgatccctggtggtcgatcacgtgcgcctgctccacttcatgacccctgaaaccatgcggtgggctactgtcctcgcctgcctgttcgccattctcctcgctatttgaagatctcccccccccctaacgttactggccgaagccgcttggaataaggccggtgtgcgtttgtctatatgttattttccaccatattgccgtcttttggcaatgtgagggcccggaaacctggccctgtcttcttgacgagcattcctaggggtctttcccctctcgccaaaggaatgcaaggtctgttgaatgtcgtgaaggaagcagttcctctggaagcttcttgaagacaaacaacgtctgtagcgaccctttgcaggcagcggaaccccccacctggcgacaggtgcctctgcggccaaaagccacgtgtataagatacacctgcaaaggcggcacaaccccagtgccacgttgtgagttggatagttgtggaaagagtcaaatggctctcctcaagcgtattcaacaaggggctgaaggatgcccagaaggtaccccattgtatgggatctgatctggggcctcggtgcacatgctttacatgtgtttagtcgaggttaaaaaacgtctaggccccccgaaccacggggacgtggttttcctttgaaaaacacgatgataataccaccatggtcaattcctgtaccttcctccacatcttcctctgttgttcattcctctattccttctgttgcgctgtcgtcgctgggtcaaacaccacatactgcttctggtttccactggtgagaggaaacttctcctttgagctcacagtcaattataccgtgtgccctccatgtctgacccgacaggcagctacagaaatctacgaacctggcaggtctctgtggtgcagaattggctatgaccgatgtggagaggacgatcacgatgaactggggttcatgatccctcccggcctgagctccgaaggacatctcacaggggtctacgcatggctggccttcctctccttttcttatactgcccagttccaccccgaaatcttcgggattggcaacgtgtccagggtgtacgtcgacatcaagcaccagctgatttgtgccgaacatgacggccagaacactaccctgcctcggcatgataatatcagcgccgtgttccagacctactatcagcaccaggtggatggcggaaattggtttcatctggagtggctccggcccttcttttcttcatggctggtcctcaacgtgtcatggttcctgcggcgcagtcccgccaatcacgtgagcgtccgggtgctgcagattctccgcccaactccacctcagaggcaggctctgctcagtagcaaaacctcagtggcactgggcatcgctacacgacctctcagacggttcgctaagtccctctcagcagtcagaaggtgaagatctggtaccgggggaggctaactgaaacacggaaggagacaataccggaaggaacccgcgctatgacggcaataaaaagacagaataaaacgcacgggtgttgggtcgtttgttcataaacgcggggttcggtcccagggctggcactctgtcgataccccaccgagaccccattggggccaatacgcccgcgtttcttccttttccccaccccaccccccaagttcgggtgaaggcccagggctcgcagccaacgtcggggcggcaggccctgccatagccagctttcttgtacaaagttggcattataagaaagcattgcttatcaatttgttgcaacgaacaggtcactatcagtcaaaataaaatcattattt

SEQ ID NO: 24 - protein, 10 aa, Artificial Sequence
  Placeholder for: vAD-rtg-gp234-E pre-recombination insert
NNNNNNNNNN

SEQ ID NO: 25 - DNA, 10 bp, Artificial Sequence
  Placeholder for: vAD3033 pre-recombination insert
  misc_feature (1)..(10): n is a, c, g, t or u
nnnnnnnnnn

SEQ ID NO: 26 - DNA, 24 bp, Artificial Sequence
  pAd5 Forward primer
gactttgaccgtttacgtggagac

SEQ ID NO: 27 - DNA, 24 bp, Artificial Sequence
  pAd5 Reverse primer
ccttaagccacgcccacacatttc

SEQ ID NO: 28 - DNA, 15411 bp, Artificial Sequence
  Entire VR2332, PRRSV Type II sequence
atgacgtataggtgttggctctatgccttggcatttgtattgtcaggagctgtgaccattggcacagcccaaaacttgctgcacagaaacacccttctgtgatagcctccttcaggggagcttagggtttgtccctagcaccttgcttccggagttgcactgctttacggtctctccacccctttaaccatgtctgggatacttgatcggtgcacgtgtacccccaatgccagggtgtttatggcggagggccaagtctactgcacacgatgcctcagtgcacggtctctccttcccctgaacctccaagtttctgagctcggggtgctaggcctattctacaggcccgaagagccactccggtggacgttgccacgtgcattccccactgttgagtgctcccccgccggggcctgctggctttctgcaatctttccaatcgcacgaatgaccagtggaaacctgaacttccaacaaagaatggtacgggtcgcagctgagctttacagagccggccagctcacccctgcagtcttgaaggctctacaagtttatgaacggggttgccgctggtaccccattgttggacctgtccctggagtggccgttttcgccaattccctacatgtgagtgataaacctttcccgggagcaactcacgtgttgaccaacctgccgctcccgcagagacccaagcctgaagacttttgcccctttgagtgtgctatggctactgtctatgacattggtcatgacgccgtcatgtatgtggccgaaaggaaagtctcctgggcccctcgtggcggggatgaagtgaaatttgaagctgtccccggggagttgaagttgattgcgaaccggctccgcacctccttcccgccccaccacacagtggacatgtctaagttcgccttcacagcccctgggtgtggtgtttctatgcgggtcgaacgccaacacggctgccttcccgctgacactgtccctgaaggcaactgctggtggagcttgtttgacttgcttccactggaagttcagaacaaagaaattcgccatgctaaccaatttggctaccagaccaagcatggtgtctctggcaagtacctacagcggaggctgcaagttaatggtctccgagcagtaactgacctaaacggacctatcgtcgtacagtacttctccgttaaggagagttggatccgccatttgaaactggcgggagaacccagctactctgggtttgaggacctcctcagaataagggttgagcctaacacgtcgccattggctgacaaggaagaaaaaattttccggtttggcagtcacaagtggtacggcgctggaaagagagcaagaaaagcacgctcttgtgcgactgctacagtcgctggccgcgctttgtccgttcgtgaaacccggcaggccaaggagcacgaggttgccggcgccaacaaggctgagcacctcaaacactactccccgcctgccgaagggaattgtggttggcactgcatttccgccatcgccaaccggatggtgaattccaaatttgaaaccacccttcccgaaagagtgagacctccagatgactgggctactgacgaggatcttgtgaatgccatccaaatcctcagactccctgcggccttagacaggaacggtgcttgtactagcgccaagtacgtacttaagctggaaggtgagcattggactgtcactgtgacccctgggatgtccccttctttgctccctcttgaatgtgttcagggctgttgtgggcacaagggcggtcttggttccccagatgcagtcgaggtctccggatttgaccctgcctgccttgaccggctggctgaggtgatgcacctgcctagcagtgctatcccagccgctctggccgaaatgtctggcgattccgatcgttcggcttctccggtcaccaccgtgtggactgtttcgcagttctttgcccgtcacagcggagggaatcaccctgaccaagtgcgcttagggaaaattatcagcctttgtcaggtgattgaggactgctgctgttcccagaacaaaaccaaccgggtcaccccggaggaggtcgcagcaaagattgacctgtacctccgtggtgcaacaaatcttgaagaatgcttggccaggcttgagaaagcgcgcccgccacgcgtaatcgacacctcctttgattgggatgttgtgctccctggggttgaggcggcaacccagacgatcaagctgccccaggtcaaccagtgtcgtgctctggtccctgttgtgactcaaaagtccttggacaacaactcggtccccctgaccgccttttcactggctaactactactaccgtgcgcaaggtgacgaagttcgtcaccgtgaaagactaaccgccgtgctctccaagttggaaaaggttgttcgagaagaatatgggctcatgccaaccgagcctggtccacggcccacactgccacgcgggctcgacgaactcaaagaccagatggaggaggacttgctgaaactggctaacgcccagacgacttcggacatgatggcctgggcagtcgagcaggttgacctaaaaacttgggtcaagaactacccgcggtggacaccaccaccccctccgccaaaagttcagcctcgaaaaacgaagcctgtcaagagcttgccggagagaaagcctgtccccgccccgcgcaggaaggttgggtccgattgtggcagcccggtttcattaggcggcgatgtccctaacagttgggaagatttggctgttagtagcccctttgatctcccgaccccacctgagccggcaacaccttcaagtgagctggtgattgtgtcctcaccgcaatgcatcttcaggccggcgacacccttgagtgagccggctccaattcccgcacctcgcggaactgtgtctcgaccggtgacacccttgagtgagccgatccctgtgcccgcaccgcggcgtaagtttcagcaggtgaaaagattgagttcggcggcggcaatcccaccgtaccaggacgagcccctggatttgtctgcttcctcacagactgaatatgaggcctctcccccagcaccgccgcagagcgggggcgttctgggagtagaggggcatgaagctgaggaaaccctgagtgaaatctcggacatgtcgggtaacattaaacctgcgtccgtgtcatcaagcagctccttgtccagcgtgagaatcacacgcccaaaatactcagctcaagccatcatcgactcgggcgggccctgcagtgggcatctccaagaggtaaaggaaacatgccttagtgtcatgcgcgaggcatgtgatgcgactaagcttgatgaccctgctacgcaggaatggctttctcgcatgtgggatcgggtggacatgctgacttggcgcaacacgtctgtttaccaggcgatttgcaccttagatggcaggttaaagttcctcccaaaaatgatactcgagacaccgccgccctatccgtgtgagtttgtgatgatgcctcacacgcctgcaccttccgtaggtgcggagagcgaccttaccattggctcagttgctactgaagatgttccacgcatcctcgagaaaatagaaaatgtcggcgagatggccaaccagggacccttggccttctccgaggataaaccggtagatgaccaacttgtcaacgacccccggatatcgtcgcggaggcctgacgagagcacatcagctccgtccgcaggcacaggtggcgccggctcttttaccgatttgccgccttcagatggcgcggatgcggacgggggggggccgtttcggacggtaaaaagaaaagctgaaaggctctttgaccaactgagccgtcaggtttttgacctcgtctcccatctccctgttttcttctcacgccttttctaccctggcggtggttattctccgggtgattggggttttgcagcttttactctattgtgcctctttttatgttacagttacccagcctttggtattgctcccctcttgggtgtgttttctgggtcttctcggcgcgttcgaatgggggtttttggctgctggttggcttttgctgttggtctgttcaagcctgtgtccgacccagtcggcgctgcttgtgagtttgactcgccagagtgtagaaacatccttcattcttttgagcttctcaaaccttgggaccctgttcgcagccttgttgtgggccccgtcggtctcggtcttgccattcttggcaggttactgggcggggcacgctgcatctggcactttttgcttaggcttggcattgttgcagactgtatcttggctggagcttacgtgctttctcaaggtaggtgtaaaaagtgctggggatcttgtataagaactgctcctaatgaggtcgcttttaacgtgtttcctttcacacgtgcgaccaggtcgtcacttatcgacctgtgcgatcggttttgtgcgccaaaaggaatggaccccatttttctcgccactgggtggcgcgggtgctgggccggccgaagccccattgagcaaccctctgaaaaacccatcgcgtttgcccaattggatgaaaagaagattacggctaggactgtggtcgcccagccttatgaccccaaccaagccgtaaagtgcttgcgggtattgcagtcgggtggggcgatggtggctaaggcggtcccaaaagtggtcaaggtttccgctgttccattccgagcccccttctttcccactggagtgaaagttgaccctgattgcagggtcgtggttgaccctgacactttcactgcagctctccggtctggctactccaccacaaacctcgtccttggtgtaggggactttgcccagctgaatggattaaaaatcaggcaaatttccaagccttcagggggaggcccacatctcatggctgccctgcatgttgcctgctcgatggctctgcacatgcttgctgggatttatgtgactgcggtgggttcttgcggcaccggcaccaacgacccgtggtgcgctaacccgtttgccgtccctggctacggacctggctctctctgcacgtccaggttgtgcatttcccaacacggccttaccctgcccttgacagcacttgtggcgggattcggtattcaagaaattgccttggtcgttttgatttttgtttccatcggaggcatggctcataggttgagctgtaaggctgacatgctgtgtgttttgcttgcaattgccagctatgtttgggtacctcttacctggttgctttgtgtgtttccttgctggttgcgctgtttttctttgcaccccctcaccatcctatggttggtgtttttcttgatttctgtgaatatgccttcaggaatcttggccatggtgttgttggtttctctttggcttcttggtcgttatactaatgttgctggccttgtcaccccctacgacattcatcattacaccagtggcccccgcggtgttgccgccttggctaccgcaccagatgggacctacttggccgctgtccgccgcgctgcgttgactggccgcaccatgctgtttaccccgtcccagcttgggtctcttcttgagggtgctttcagaactcgaaagccctcactgaacaccgtcaatgtgatcgggtcctccatgggctctggcggggtgtttaccatcgacgggaaagtcaagtgcgtaactgccgcacatgtccttacgggcaattcagctcgggtttccggggtcggcttcaatcaaatgcttgactttgacgtaaagggagatttcgctatagctgattgcccgaattggcaaggggctgcccccaagacccaattctgcacggatggatggactggccgtgcctattggctaacatcctctggcgtcgaacccggcgtcattggaaaaggattcgccttctgcttcaccgcatgtggcgattccgggtccccagtgatcaccgaggccggtgagcttgtcggcgttcacacgggatcgaataaacaaggggggggcattgttacgcgcccctcaggccagttttgtaatgtggcacccatcaagctaagcgaattaagtgaattctttgctgggcctaaggtcccgctcggtgatgtgaaggtcggcagccacataattaaagacataagcgaggtgccttcagatctttgtgccttgcttgctgccaaacctgaactggaaggaggcctctccaccgtccaacttctttgtgtgttttttctcctgtggagaatgatgggacatgcctggacgcccttggttgctgtgagtttctttattttgaatgaggttctcccagccgtcctggtccggagtgttttctcctttggaatgtttgtgctatcctggctcacgccatggtctgcgcaagttctgatgatcaggcttctgacagcagctcttaacaggaacagatggtcacttgcctttttcagcctcggtgcagtgaccggttttgtcgcagatcttgcggccactcaggggcatccgttgcaggcagtgatgaatttgagcacctatgcattcctgcctcggatgatggttgtgacctcaccagtcccagtgatcacgtgtggtgtcgtgcacctacttgccatcattttgtacttgtttaagtaccgtggcccgcaccatatccttgttggcgatggagtgttctctgcggctttcttcttgagatactttgccgagggaaagttgagggaaggggtgtcgcaatcctgcggaatgaatcatgagtctctgactggtgccctcgctatgagactcaatgacgaggacttggatttccttatgaaatggactgattttaagtgctttgtttctgcgtccaacatgaggaatgcagcgggtcaatttatcgaggctgcctatgctaaagcacttagagtagaactggcccagttggtgcaggttgataaagttcgaggtactttggccaaacttgaagcttttgctgataccgtggcacctcaactctcgcccggtgacattgttgtcgctctcggccacacgcctgttggcagtatcttcgacctaaaggttggtagcaccaagcataccctccaagccattgagaccagagtccttgctgggtccaaaatgaccgtggcgcgcgtcgtcgacccgacccccacgcccccacccgcacccgtgcccatccccctcccaccgaaagttctggagaatggccccaacgcttggggggatgaggaccgtttgaataagaagaagaggcgcaggatggaagccctcggcatctatgttatgggcgggaaaaagtaccagaaattttgggacaagaattccggtgatgtgttttatgaggaggtccataataacacagatgagtgggagtgtctcagagttggcgaccctgccgactttgaccctgagaagggaactctgtgtggacatgtcaccattgaaaacaaggcttaccatgtttacacctccccatctggtaagaagttcttggtccccgtcaacccagagaatggaagagttcaatgggaagctgcaaagctttccgtggagcaggccctaggtatgatgaatgtcgacggcgaactgactgccaaagaactggagaaactgaaaagaataattgacaaactccagggcctgactaaggagcagtgtttaaactgctagccgccagcgacttgacccgctgtggtcgcggcggcttggttgttactgaaacagcggtaaaaatagtcaaatttcacaaccggaccttcaccctgggacctgtgaatttaaaagtggccagtgaggttgagctaaaagacgcggttgagcacaaccaacacccggttgcgagaccgatcgatggtggagttgtgctcctgcgttccgcggttccttcgcttatagacgtcttgatctccggtgctgatgcatctcccaagttacttgcccatcacgggccgggaaacactgggatcgatggcacgctctgggattttgagtccgaagccactaaagaggaagtcgcactcagtgcgcaaataatacaggcttgtgacattaggcgcggcgacgctcctgaaattggtctcccttacaagctgtaccctgttaggggtaaccctgagcgggtgaaaggagttctgcagaatacaaggtttggagacataccttacaaaacccccagtgacactggaagcccagtgcacgcggctgcctgccttacgcccaacgccactccggtgactgatgggcgctccgtcttggccacgaccatgccccccgggtttgagttatatgtaccgaccataccagcgtctgtccttgattaccttgactctaggcctgactgccctaaacagctgacagagcacggctgcgaagatgccgcactgaaagacctctctaaatatgacttgtccacccaaggctttgttttacctggagttcttcgccttgtgcggaaatacctgtttgcccatgtaggtaagtgcccacccgttcatcggccttctacttaccctgctaagaattctatggctggaataaatgggaacaggttcccaaccaaggacattcagagcgtccctgaaatcgacgttctgtgcgcacaggctgtgcgagaaaactggcaaactgtcaccccttgtactcttaagaaacagtattgcgggaagaagaagactaggaccatactcggcaccaataacttcatcgcactagcccaccgagcagtgttgagtggtgttacccagggcttcatgaaaaaggcgtttaactcgcccatcgccctcggaaagaacaagtttaaggagctacagactccggtcctgggcaggtgccttgaagctgatctcgcatcctgcgatcgatccacgcctgcaattgtccgctggtttgccgccaaccttctttatgaacttgcctgtgctgaagagcatctaccgtcgtacgtgctgaactgctgccacgacttactggtcacgcagtccggcgcagtgactaagagaggtggcctgtcgtctggcgacccgatcacctctgtgtctaacaccatttatagtttggtgatctatgcacagcatatggtgcttagttacttcaaaagtggtcacccccatggccttctgttcttacaagaccagctaaagtttgaggacatgctcaaggttcaacccctgatcgtctattcggacgacctcgtgctgtatgccgagtctcccaccatgccaaactatcactggtgggttgaacatctgaatttgatgctggggtttcagacggacccaaagaagacagcaataacagactcgccatcatttctaggctgtagaataataaatgggcgccagctagtccccaaccgtgacaggatcctcgcggccctcgcctatcacatgaaggcgagtaatgtttctgaatactatgcctcagcggctgcaatactcatggacagctgtgcttgtttggagtatgatcctgaatggtttgaagaacttgtagttggaatagcgcagtgcgcccgcaaggacggctacagctttcccggcacgccgttcttcatgtccatgtgggaaaaactcaggtccaattatgaggggaagaagtcgagagtgtgcgggtactgcggggccccggccccgtacgctactgcctgtggcctcgacgtctgcatttaccacacccacttccaccagcattgtccagtcacaatctggtgtggccatccagcgggttctggttcttgtagtgagtgcaaatcccctgtagggaaaggcacaagccctttagacgaggtgctggaacaagtcccgtataagcccccacggaccgttatcatgcatgtggagcagggtctcaccccccttgatccaggtagataccaaactcgccgcggattagtctctgtcaggcgtggaattaggggaaatgaagttggactaccagacggtgattatgctagcaccgccttgctccctacctgcaaagagatcaacatggtcgctgtcgcttccaatgtattgcgcagcaggttcatcatcggcccacccggtgctgggaaaacatactggctccttcaacaggtccaggatggtgatgttatttacacaccaactcaccagaccatgcttgacatgattagggctttggggacgtgccggttcaacgtcccggcaggcacaacgctgcaattccccgtcccctcccgcaccggtccgtgggttcgcatcctagccggcggttggtgtcctggcaagaattccttcctagatgaagcagcgtattgcaatcaccttgatgttttgaggcttcttagtaaaactaccctcacctgtctaggagacttcaagcaactccacccagtgggttttgattctcattgctatgtttttgacatcatgcctcaaactcaactgaagaccatctggaggtttggacagaatatctgtgatgccattcagccagattacagggacaaactcatgtccatggtcaacacaacccgtgtgacctacgtggaaaaacctgtcaggtatgggcaggtcctcaccccctaccacagggaccgagaggacgacgccatcactattgactccagtcaaggcgccacattcgatgtggttacattgcatttgcccactaaagattcactcaacaggcaaagagcccttgttgctatcaccagggcaagacacgctatctttgtgtatgacccacacaggcagctgcagggcttgtttgatcttcctgcaaaaggcacgcccgtcaacctcgcagtgcactgcgacgggcagctgatcgtgctggatagaaataacaaagaatgcacggttgctcaggctctaggcaacggggataaatttagggccacagacaagcgtgttgtagattctctccgcgccatttgtgctgatctagaagggtcgagctctccgctccccaaggtcgcacacaacttgggattttatttctcacctgatttaacacagtttgctaaactcccagtagaacttgcacctcactggcccgtggtgtcaacccagaacaatgaaaagtggccggatcggctggttgccagccttcgccctatccataaatacagccgcgcgtgcatcggtgccggctatatggtgggcccttcggtgtttctaggcactcctggggtcgtgtcatactatctcacaaaatttgttaagggcggggctcaagtgcttccggagacggttttcagcaccggccgaattgaggtagactgccgggaatatcttgatgatcgggagcgagaagttgctgcgtccctcccacacggtttcattggcgacgtcaaaggcactaccgttggaggatgtcatcatgtcacctccagatacctcccgcgcgtccttcccaaggaatcagttgcggtagtcggggtttcaagccccggaaaagccgcgaaagcattgtgcacactgacagatgtgtacctcccagatcttgaagcctatctccacccggagacccagtccaagtgctggaaaatgatgttggacttcaaagaagttcgactaatggtctggaaagacaaaacagcctatttccaacttgaaggtcgctatttcacctggtatcagcttgccagctatgcctcgtacatccgtgttcccgtcaactctacggtgtacttggacccctgcatgggccccgccctttgcaacaggagagtcgtcgggtccacccactggggggctgacctcgcggtcaccccttatgattacggcgctaaaattatcctgtctagcgcgtaccatggtgaaatgccccccggatacaaaattctggcgtgcgcggagttctcgttggatgacccagttaagtacaaacatacctgggggtttgaatcggatacagcgtatctgtatgagttcaccggaaacggtgaggactgggaggattacaatgatgcgtttcgtgcgcgccaggaagggaaaatttataaggccactgccaccagcttgaagttttattttcccccgggccctgtcattgaaccaactttaggcctgaattgaaatgaaatggggtccatgcaaagcctttttgacaaaattggccaactttttgtggatgctttcacggagttcttggtgtccattgttgatatcattatatttttggccattttgtttggcttcaccatcgccggttggctggtggtcttttgcatcagattggtttgctccgcgatactccgtacgcgccctgccattcactctgagcaattacagaagatcttatgaggcctttctttcccagtgccaagtggacattcccacctggggaactaaacatcctttggggatgctttggcaccataaggtgtcaaccctgattgatgaaatggtgtcgcgtcgaatgtaccgcatcatggaaaaagcagggcaggctgcctggaaacaggtggtgagcgaggctacgctgtctcgcattagtagtttggatgtggtggctcattttcagcatctagccgccattgaagccgagacctgtaaatatttggcctcccggctgcccatgctacacaacctgcgcatgacagggtcaaatgtaaccatagtgtataatagcactttgaatcaggtgtttgctatttttccaacccctggttcccggccaaagcttcatgattttcagcaatggttaatagctgtacattcctccatattttcctctgttgcagcttcttgtactctttttgttgtgctgtggttgcgggttccaatactacgtactgtttttggtttccgctggttaggggcaatttttctttcgaactcacagtgaattacacggtgtgtccaccttgcctcacccggcaagcagccacagagatctacgaacccggtaggtctctttggtgcaggatagggtatgaccgatgtggggaggacgatcatgacgagctagggtttatgataccgcctggcctctccagcgaaggccacttgactggtgtttacgcctggttggcgttcttgtccttcagctacacggcccagttccatcccgagatattcgggatagggaatgtgagtcgagtttatgttgacatcaaacatcaactcatctgcgccgaacatgacgggcagaacaccaccttgcctcgtcatgacaacatttcagccgtgtttcagacctattaccaacatcaagtcgacggcggcaattggtttcacctagaatggcttcgtcccttcttttcctcgtggttggttttaaatgtctcttggtttctcaggcgttcgcctgcaaaccatgtttcagttcgagtcttgcagatattaagaccaacaccaccgcagcggcaagctttgctgtcctccaagacatcagttgccttaggcatcgcgactcggcctctgaggcgattcgcaaaatccctcagtgccgtacggcgatagggacacccgtgtatgttaccatcacagccaatgtgacagatgagaattatttacattcttctgatctcctcatgctttcttcttgccttttctatgcttctgagatgagtgaaaagggatttaaggtggtatttggcaatgtgtcaggcatcgtggctgtgtgtgtcaattttaccagctacgtccaacatgtcaaggagtttacccaacgctccctggtggtcgaccatgtgcggttgctccatttcatgacacctgagaccatgaggtgggcaactgttttagcctgtctttttgccattctgttggcaatttgaatgtttaagtatgttggagaaatgcttgaccgcgggctgttgctcgcgattgctttctttgtggtgtatcgtgccgttctgttttgctgtgctcgccaacgccagcaacgacagcagctcccatctacagctgatttacaacttgacgctatgtgagctgaatggcacagattggctagctaacaaatttgattgggcagtggagagttttgtcatctttcccgttttgactcacattgtctcctatggtgccctcactaccagccatttccttgacacagtcgctttagtcactgtgtctaccgccgggtttgttcacgggcggtatgtcctaagtagcatctacgcggtctgtgccctggctgcgttgacttgcttcgtcattaggtttgcaaagaattgcatgtcctggcgctacgcgtgtaccagatataccaactttcttctggacactaagggcagactctatcgttggcggtcgcctgtcatcatagagaaaaggggcaaagttgaggtcgaaggtcatctgatcgacctcaaaagagttgtgcttgatggttccgtggcaacccctataaccagagtttcagcggaacaatggggtcgtccttagatgacttctgtcatgatagcacggctccacaaaaggtgcttttggcgttttctattacctacacgccagtgatgatatatgccctaaaggtgagtcgcggccgactgctagggcttctgcaccttttgatcttcctgaattgtgctttcaccttcgggtacatgactttcgcgcactttcagagtacaaataaggtcgcgctcactatgggagcagtagttgcactcctttggggggtgtactcagccatagaaacctggaaattcatcacctccagatgccgtttgtgcttgctaggccgcaagtacattctggcccctgcccaccacgttgaaagtgccgcacggtttcatccgattgcggcaaatgataaccacgcatttgtcgtccggcgtcccggctccactacggtcaacggcacattggtgcccgggttaaaaagcctcgtgttgggtggcagaaaagctgttaaacagggagtggtaaaccttgtcaaatatgccaaataacaacggcaagcagcagaagagaaagaagggggatggccagccagtcaatcagctgtgccagatgctgggtaagatcatcgctcagcaaaaccagtccagaggcaagggaccgggaaagaaaaataagaagaaaaacccggagaagccccattttcctctagcgactgaagatgatgtcagacatcactttacccctagtgagcggcaattgtgtctgtcgtcaatccagaccgcctttaatcaaggcgctgggacttgcaccctgtcagattcagggaggataagttacactgtggagtttagtttgcctacgcatcatactgtgcgcctgatccgcgtcacagcatcaccctcagcatgatgggctggcattcttgaggcatctcagtgtttgaattggaagaatgtgtggtgaatggcactgattgacattgtgcctctaagtcacctattcaattagggcgaccgtgtgggggtgagatttaattggcgagaaccatgcggccgaaatt

SEQ ID NO: 29 - DNA, 15108 bp, Artificial Sequence
  Entire Lelystad PRRSV sequence (GenBank: A26843.1)
gggtattccccctacatacacgacacttctagtgtttgtgtaccttggaggcgtgggtacagccccgccccaccccttggcccctgttctagcccaacaggtatccttctctctcggggcgagtgcgccgcctgctgctcccttgcagcgggaaggacctcccgagtatttccggagagcacctgctttacgggatctccaccctttaaccatgtctgggacgttctcccggtgcatgtgcaccccggctgcccgggtattttggaacgccggccaagtcttttgcacacggtgtctcagtgcgcggtctcttctctctccagagcttcaggacactgacctcggtgcagttggcttgttttacaagcctagggacaagcttcactggaaagtccctatcggcatccctcaggtggaatgtactccatccgggtgctgttggctctcagctgttttccctttggcgcgtatgacctccggcaatcacaacttcctccaacgacttgtgaaggttgctgatgttttgtaccgtgacggttgcttggcacctcgacaccttcgtgaactccaagtttacgagcgcggctgcaactggtacccgatcacggggcccgtgcccgggatgggtttgtttgcgaactccatgcacgtatccgaccagccgttccctggtgccacccatgtgttgactaactcgcctttgcctcaacaggcttgtcggcagccgttctgtccatttgaggaggctcattctagcgtgtacaggtggaagaaatttgtggttttcacggactcctccctcaacggtcgatctcgcatgatgtggacgccggaatccgatgattcagccgccctggaggtactaccgcctgagttagaacgtcaggtcgaaatcctcattcggagttttcctgctcatcaccctgtcgacctggccgactgggagctcactgagtcccctgagaacggtttttccttcaacacgtctcattcttgcggtcaccttgtccagaaccccgacgtgtttgatggcaagtgctggctctcctgctttttgggccagtcggtcgaagtgcgctgccatgaggaacatctagctgacgccttcggttaccaaaccaagtggggcgtgcatggtaagtacctccagcgcaggcttcaagttcgcggcattcgtgctgtagtcgatcctgatggtcccattcacgttgaagcgctgtcttgcccccagtcttggatcaggcacctgactctggatgatgatgtcaccccaggattcgttcgcctgacatcccttcgcattgtgccgaacacagagcctaccacttcccggatctttcggtttggagcgcataagtggtatggcgctgccggcaaacgggctcgtgctaagcgtgccgctaaaagtgagaaggattcggctcccacccccaaggttgccctgccggtccccacctgtggaattaccacctactctccaccgacagacgggtcttgtggttggcatgtccttgccgccataatgaaccggatgataaatggtgacttcacgtcccctctgactcagtacaacagaccagaggatgattgggcttctgattatgatcttgttcaggcgattcaatgtctacgactgcctgctaccgtggttcggaatcgcgcctgtcctaacgccaagtaccttataaaacttaacggagttcactgggaggtagaggtgaggtctggaatggctcctcgctccctttctcgtgaatgtgtggttggcgtttgctctgaaggctgtgtcgcaccgccttatccagcagacgggctacctaaacgtgcactcgaggccttggcgtctgcttacagactaccctccgattgtgttagctctggtattgctgactttcttgctaatccacctcctcaggaattctggaccctcgacaaaatgttgacctccccgtcaccagagcggtccggcttctctagtttgtataaattactattagaggttgttccgcaaaaatgcggtgccacggaaggggctttcatctatgctgttgagaggatgttgaaggattgtccgagctccaaacaggccatggcccttctggcaaaaattaaagttccatcctcaaaggccccgtctgtgtccctggacgagtgtttccctacggatgttttagccgacttcgagccagcatctcaggaaaggccccaaagttccggcgctgctgttgtcctgtgttcaccggatgcaaaagagttcgaggaagcagccccggaagaagttcaagagagtggccacaaggccgtccactctgcactccttgccgagggtcctaacaatgagcaggtacaggtggttgccggtgagcaactgaagctcggcggttgtggtttggcagtcgggaatgctcatgaaggtgctctggtctcagctggtctaattaacctggtaggcgggaatttgtccccctcagaccccatgaaagaaaacatgctcaatagccgggaagacgaaccactggatttgtcccaaccagcaccagcttccacaacgacccttgtgagagagcaaacacccgacaacccaggttctgatgccggtgccctccccgtcaccgttcgagaatttgtcccgacggggcctatactctgtcatgttgagcactgcggcacggagtcgggcgacagcagttcgcctttggatctatctgatgcgcaaaccctggaccagcctttaaatctatccctggccgcttggccagtgagggccaccgcgtctgaccctggctgggtccacggtaggcgcgagcctgtctttgtaaagcctcgaaatgctttctctgatggcgattcagcccttcagttcggggagctttctgaatccagctctgtcatcgagtttgaccggacaaaagatgctccggtggttgacgcccctgtcgacttgacgacttcgaacgaggccctctctgtagtcgatcctttcgaatttgccgaactcaagcgcccgcgtttctccgcacaagccttaattgaccgaggcggtccacttgccgatgtccatgcaaaaataaagaaccgggtatatgaacagtgcctccaagcttgtgagcccggtagtcgtgcaaccccagccaccagggagtggctcgacaaaatgtgggatagggtggacatgaaaacttggcgctgcacctcgcagttccaagctggtcgcattcttgcgtccctcaaattcctccctgacatgattcaagacacaccgcctcctgttcccaggaagaaccgagctagtgacaatgccggcctgaagcaactggtggcacagtgggataaggaaattgagtgtgacccccccccaaaaccggttgggccagtgcttgaccagatcgtccctccgcctacggatatccagcaagaagatgtcaccccctccgatgggccaccccatgcgccggattttcctagtcgagtgagcacgggcgggagttggaaaggccttatgctttccggcacccgtctcgcggggtctatcagccagcgccttatgacatgggtttttgaagttttctcccacctcccagcttttatgctcacacttttctcgccgcggggctctatggctccaggtgattggttgtttgcaggtgtcgttttacttgctctcttgctctgtcgttcttacccgatactcggatgccttcccttattgggtgtcttttctggttctttgcggcgtgttcgtctgggtgtttttggttcttggatggcttttgctgtatttttattctcgactccatccaacccagtcggttcttcttgtgaccacgattcgccggagtgtcatgctgagcttttggctcttgagcagcgccaactttgggaacctgtgcgcggccttgtggtcggcccctcaggcctcttatgtgtcattcttggcaagttactcggtgggtcacgttatctctggcatgttctcctacgtttatgcatgcttgcagatttggccctttctcttgtttatgtggtgtcccaggggcgttgtcacaagtgttggggaaagtgtataaggacagctcctgcggaggtggctcttaatgtatttcctttctcgcgcgccacccgtgtctctcttgtatccttgtgtgatcgattccaaacgccaaaaggggttgatcctgtgcacttggcaacgggttggcgcgggtgctggcgtggtgagagccccatccatcaaccacaccaaaagcccatagcttatgccaatttggatgaaaagaaaatgtctgcccaaacggtggttgctgtcccatacgatcccagtcaggctatcaaatgcctgaaagttctgcaggcgggaggggccatcgtggaccagcctacacctgaggtcgttcgtgtgtccgagatccccttctcagccccatttttcccaaaagttccagtcaacccagattgcagggttgtggtagattcggacacttttgtggctgcggttcgctgcggttactcgacagcacaactggttctgggccggggcaactttgccaagttaaatcagaccccccccaggaactctatctccaccaaaacgactggtggggcctcttacacccttgctgtggctcaagtgtctgcgtggactcttgttcatttcatcctcggtctttggttcacatcacctcaagtgtgtggccgaggaaccgctgacccatggtgttcaaatcctttttcatatcctacctatggccccggagttgtgtgctcctctcgactttgtgtgtctgccgacggggtcaccctgccattgttctcagccgtggcacaactctccggtagagaggtggggatttttattttggtgctcgtctccttgactgctttggcccaccgcatggctcttaaggcagacatgttagtggtcttttcggctttttgtgcttacgcctggcccatgagctcctggttaatctgcttctttcctatactcttgaagtgggttacccttcaccctcttactatgctttgggtgcactcattcttggtgttttgtctgccagcagccggcatcctctcactagggataactggccttctttgggcaattggccgctttacccaggttgccggaattattacaccttatgacatccaccagtacacctctgggccacgtggtgcagctgctgtggccacagccccagaaggcacttatatggccgccgtccggagagctgctttaactgggcgaactttaatcttcaccccgtctgcagttggatcccttctcgaaggtgctttcaggactcataaaccctgccttaacaccgtgaatgttgtaggctcttcccttggttccggaggggttttcaccattgatggcagaagaactgtcgtcactgctgcccatgtgttgaacggcgacacagctagagtcaccggcgactcctacaaccgcatgcacactttcaagaccaatggtgattatgcctggtcccatgctgatgactggcagggcgttgcccctgtggtcaaggttgcgaaggggtaccgcggtcgtgcctactggcaaacatcaactggtgtcgaacccggtatcattggggaagggttcgccttctgttttactaactgcggcgattcggggtcacccgtcatctcagaatctggtgatcttattggaatccacaccggttcaaacaaacttggttctggtcttgtgacaacccctgaaggggagacctgcaccatcaaagaaaccaagctctctgacctttccagacattttgcaggcccaagcgttcctcttggggacattaaattgagtccggccatcatccctgatgtaacatccattccgagtgacttggcatcgctcctagcctccgtccctgtagtggaaggcggcctctcgaccgttcaacttttgtgtgtctttttccttctctggcgcatgatgggccatgcctggacacccattgttgccgtgggcttctttttgctgaatgaaattcttccagcagttttggtccgagccgtgttttcttttgcactctttgtgcttgcatgggccaccccctggtctgcacaggtgttgatgattagactcctcacggcatctctcaaccgcaacaagctttctctggcgttctacgcactcgggggtgtcgtcggtttggcagctgaaatcgggacttttgctggcagattgtctgaattgtctcaagctctttcgacatactgcttcttacctagggtccttgctatgaccagttgtgttcccaccatcatcattggtggactccataccctcggtgtgattctgtggttattcaaataccggtgcctccacaacatgctggttggtgatgggagtttttcaagcgccttcttcctacggtattttgcagagggtaatctcagaaaaggtgtttcacagtcctgtggcatgaataacgagtccctaacggctgctttagcttgcaagttgtcacaggctgaccttgattttttgtccagcttaacgaacttcaagtgctttgtatctgcttcaaacatgaaaaatgctgccggccagtacattgaagcagcgtatgccaaggccctgcgccaagagttggcctctctagttcagattgacaaaatgaaaggagttttgtccaagctcgaggcctttgctgaaacagccaccccgtcccttgacataggtgacgtgattgttctgcttgggcaacatcctcacggatccatcctcgatattaatgtggggactgaaaggaaaactgtgtccgtgcaagagacccggagcctaggcggctccaaattcagtgtttgtactgtcgtgtccaacacacccgtggacgccttgaccggcatcccactccagacaccaacccctctttttgagaatggtccgcgtcatcgcagcgaggaagacgatcttaaagtcgagaggatgaagaaacactgtgtatccctcggcttccacaacatcaatggcaaagtttactgcaaaatttgggacaagtctaccggtgacaccttttacacggatgattcccggtacacccaagaccatgcttttcaggacaggtcagccgactacagagacagggactatgagggtgtgcaaaccaccccccaacagggatttgatccaaagtctgaaacccctgttggcactgttgtgatcggcggtattacgtataacaggtatctgatcaaaggtaaggaggttctggtccccaagcctgacaactgccttgaagctgccaagctgtcccttgagcaagctctcgctgggatgggccaaacttgcgaccttacagctgccgaggtggaaaagctaaagcgcatcattagtcaactccaaggtttgaccactgaacaggctttaaactgttagccgccagcggcttgacccgctgtggccgcggcggcctagttgtgactgaaacggcggtaaaaattataaaataccacagcagaactttcaccttaggccctttagacctaaaagtcacttccgaggtggaggtaaagaaatcaactgagcagggccacgctgttgtggcaaacttatgttccggtgtcatcttgatgagacctcacccaccgtcccttgtcgacgttcttctgaaacccggacttgacacaatacccggcattcaaccagggcatggggccgggaatatgggcgtggacggttctatttgggattttgaaaccgcacccacaaaggcagaactcgagttatccaagcaaataatccaagcatgtgaagttaggcgcggggacgccccgaacctccaactcccttacaagctctatcctgttaggggggatcctgagcggcataaaggccgccttatcaataccaggtttggagatttaccttacaaaactcctcaagacaccaagtccgcaatccacgcggcttgttgcctgcaccccaacggggcccccgtgtctgatggtaaatccacactaggtaccactcttcaacatggtttcgagctttatgtccctactgtgccctatagtgtcatggagtaccttgattcacgccctgacaccccttttatgtgtactaaacatggcacttccaaggctgctgcagaggacctccaaaaatacgacctatccacccaaggatttgtcctgcctggggtcctacgcctagtacgcagattcatctttggccatattggtaaggcgccgccattgttcctcccatcaacctatcccgccaagaactctatggcagggatcaatggccagaggttcccaacaaaggacgttcagagcatacctgaaattgatgaaatgtgtgcccgcgctgtcaaggagaattggcaaactgtgacaccttgcaccctcaagaaacagtactgttccaagcccaaaaccaggaccatcctgggcaccaacaactttattgccttggctcacagatcggcgctcagtggtgtcacccaggcattcatgaagaaggcttggaagtccccaattgccttggggaaaaacaaattcaaggagctgcattgcactgtcgccggcaggtgtcttgaggccgacttggcctcctgtgaccgcagcacccccgccattgtaagatggtttgttgccaacctcctgtatgaacttgcaggatgtgaagagtacttgcctagctatgtgcttaattgctgccatgacctcgtggcaacacaggatggtgccttcacaaaacgcggtggcctgtcgtccggggaccccgtcaccagtgtgtccaacaccgtatattcactggtaatttatgcccagcacatggtattgtcggccttgaaaatgggtcatgaaattggtcttaagttcctcgaggaacagctcaagttcgaggacctccttgaaattcagcctatgttggtatactctgatgatcttgtcttgtacgctgaaagacccacatttcccaattaccactggtgggtcgagcaccttgacctgatgctgggtttcagaacggacccaaagaaaaccgtcataactgataaacccagcttcctcggctgcagaattgaggcagggcgacagctagtccccaatcgcgaccgcatcctggctgctcttgcatatcacatgaaggcgcagaacgcctcagagtattatgcgtctgctgccgcaatcctgatggattcatgtgcttgcattgaccatgaccctgagtggtatgaggacctcatctgcggtattgcccggtgcgcccgccaggatggttatagcttcccaggtccggcatttttcatgtccatgtgggagaagctgagaagtcataatgaagggaagaaattccgccactgcggcatctgcgacgccaaagccgactatgcgtccgcctgtgggcttgatttgtgtttgttccattcgcactttcatcaacactgccctgtcactctgagctgcggtcaccatgccggttcaaaggaatgttcgcagtgtcagtcacctgttggggctggcagatcccctcttgatgccgtgctaaaacaaattccatacaaacctcctcgtactgtcatcatgaaggtgggtaataaaacaacggccctcgatccggggaggtaccagtcccgtcgaggtctcgttgcagtcaagaggggtattgcaggcaatgaagttgatctttctgatggggactaccaagtggtgcctcttttgccgacttgcaaagacataaacatggtgaaggtggcttgcaatgtactactcagcaagttcatagtagggccaccaggttccggaaagaccacctggctactgagtcaagtccaggacgatgatgtcatttacacacccacccatcagactatgtttgatatagtcagtgctctcaaagtttgcaggtattccattccaggagcctcaggactccctttcccaccacctgccaggtccgggccgtgggttaggcttattgccagcgggcacgtccctggccgagtatcatacctcgatgaggctggatattgtaatcatctggacattcttagactgctttccaaaacaccccttgtgtgtttgggtgaccttcagcaacttcaccctgtcggctttgattcctactgttatgtgttcgatcagatgcctcagaagcagctgaccactatttacagatttggccctaacatctgcgcacgcatccagccttgttacagggagaaacttgaatctaaggctaggaacactagggtggtttttaccacccggcctgtggcctttggtcaggtgctgacaccataccataaagatcgcatcggctctgcgataaccatagattcatcccagggggccacctttgatattgtgacattgcatctaccatcgccaaagtccctaaataaatcccgagcacttgtagccatcactcgggcaagacacgggttgttcatttatgaccctcataaccagctccaggagtttttcaacttaacccctgagcgcactgattgtaaccttgtgttcagccgtggggatgagctggtagttctgaatgcggataatgcagtcacaactgtagcgaaggcccttgagacaggtccatctcgatttcgagtatcagacccgaggtgcaagtctctcttagccgcttgttcggccagtctggaagggagctgtatgccactaccgcaagtggcacataacctggggttttacttttccccggacagtccaacatttgcacctctgccaaaagagttggcgccacattggccagtggttacccaccagaataatcgggcgtggcctgatcgacttgtcgctagtatgcgcccaattgatgcccgctacagcaagccaatggtcggtgcagggtatgtggtcagtatgcgcccaattgatgcccgctacagcaagccaatggtcggtgcagggtatgtggtcaggggtgagccccaggccttgccagaaacactcgtttcaacagggcgtatagccacagattgtcgggagtatctcgacgcggctgaggaagaggcagcaaaagaactcccccacgcattcattggcgatgtcaaaggtaccacggttggggggtgtcatcacattacatcaaaatacctacctaggtccctgcctaaggactctgttgccgtagttggagtaagttcgcccggcagggctgctaaagccgtgtgcactctcaccgatgtgtacctccccgaactccggccatatctgcaacctgagacggcatcaaaatgctggaaactcaaattagacttcagggacgtccgactaatggtctggaaaggagccaccgcctatttccagttggaagggcttacatggtcggcgctgcccgactatgccaggtttattcagctgcccaaggatgccgttgtatacattgatccgtgtataggaccggcaacagccaaccgtaaggtcgtgcgaaccacagactggcgggccgacctggcagtgacaccgtatgattacggtgcccagaacattttgacaacagcctggttcgaggacctcgggccgcagtggaagattttggggttgcagccctttaggcgagcatttggctttgaaaacactgaggattgggcaatccttgcacgccgtatgaatgacggcaaggactacactgactataactggaactgtgttcgagaacgcccacacgccatctacgggcgtgctcgtgaccatacgtatcattttgcccctggcacagaattgcaggtagagctaggtaaaccccggctgccgcctgggcaagtgccgtgaattcggggtgatgcaatggggtcactgtggagtaaaatcagccagctgttcgtggacgccttcactgagttccttgttagtgtggttgatattgccattttccttgccatactgtttgggttcaccgtcgcaggatggttactggtctttcttctcagagtggtttgctccgcgcttctccgttcgcgctctgccattcactctcccgaactatcgaaggtcctatgaaggcttgttgcccaactgcagaccggatgtcccacaatttgcagtcaagcacccattgggyatgttttggcacatgcgagtttcccacttgattgatgagatggtctctcgtcgcatttaccagaccatggaacattcaggtcaagcggcctggaagcaggtggttggtgaggccactctcacgaagctgtcagggctcgatatagttactcatttccaacacctggccgcagtggaggcggattcttgccgctttctcagctcacgactcgtgatgctaaaaaatcttgccgttggcaatgtgagcctacagtacaacaccacgttggaccgcgttgagctcatcttccccacgccaggtacgaggcccaagttgaccgatttcagacaatggctcatcagtgtgcacgcttccattttttcctctgtggcttcatctgttaccttgttcatagtgctttggcttcgaattccagctctacgctatgtttttggtttccattggcccacggcaacacatcattcgagctgaccatcaactacaccatatgcatgccctgttctaccagtcaagcggctcgccaaaggctcgagcccggtcgtaacatgtggtgcaaaatagggcatgacaggtgtgaggagcgtgaccatgatgagttgttaatgtccatcccgtccgggtacggacaactcaaacttgagggttattatgcttggctggcttttttgtccttttcctacgcggcccaattccatccggagttgttcgggatagggaatgtgtcgcgcgtcttcgtggacaagcgacaccagttcatttgtgccgagcatgatggacacaattcaaccgtatctaccggacacaacatctccgcattatatgcggcatattaccaccaccaaatagacgggggcaattggttccatttggaatggctgcggccactcttttcttcctggctggtgctcaacatatcatggtttctgaggcgttcgcctgtaagccctgtttctcgacgcatctatcagatattgagaccaacacgaccgcggctgccggtttcatggtccttcaggacatcaattgtttccgacctcacggggtctcagcagcgcaagagaaaatttccttcggaaagtcgtcccaatgtcgtgaagccgtcggtactccccagtacatcacgataacggctaacgtgaccgacgaatcatacttgtacaacgcggacctgctgatgctttctgcgtgccttttctacgcctcagaaatgagcgagaaaggcttcaaagtcatctttgggaatgtctctggcgttgtttctgcttgtgtcaatttcacagattatgtggcccatgtgacccaacatacccagcagcatcatctggtaattgatcacattcggttgctgcatttcctgacaccatctgcaatgaggtgggctacaaccattgcttgtttgttcgccattctcttggcaatatgagatgttctcacaaattggggcgtttcttgactccgcactcttgcttctggtggctttttttgctgtgtaccggcttgtcctggtcctttgccgatggcaacggcgacagctcgacataccaatacatatataacttgacgatatgcgagctgaatgggaccgactggttgtccagccattttggttgggcagtcgagacctttgtgctttacccggttgccactcatatcctctcactgggttttctcacaacaagccatttttttgacgcgctcggtctcggcgctgtatccactgcaggatttgttggcgggcggtacgtactctgcagcgtctacggcgcttgtgctttcgcagcgttcgtatgttttgtcatccgtgctgctaaaaattgcatggcctgccgctatgcccgtacccggtttaccaacttcattgtggacgaccgggggagagttcatcgatggaagtctccaatagtggtagaaaaattgggcaaagccgaagtcgatggcaacctcgtcaccatcaaacatgtcgtcctcgaaggggttaaagctcaacccttgacgaggacttcggctgagcaatgggaggcctagacgatttttgcaacgatcctatcgccgcacaaaagctcgtgctagcctttagcatcacatacacacctataatgatatacgcccttaaggtgtcacgcggccgactcctggggctgttgcacatcctaatatttctgaactgttcctttacattcggatacatgacatatgtgcattttcaatccaccaaccgtgtcgcacttaccctgggggctgttgtcgcccttctgtggggtgtttacagcttcacagagtcatggaagtttatcacttccagatgcagattgtgttgccttggccggcgatacattctggcccctgcccatcacgtagaaagtgctgcaggtctccattcaatctcagcgtctggtaaccgagcatacgctgtgagaaagcccggactaacatcagtgaacggcactctagtaccaggacttcggagcctcgtgctgggcggcaaacgagctgttaaacgaggagtggttaacctcgtcaagtatggccggtaaaaaccagagccagaagaaaaagaaaagtacagctccgatggggaatggccagccagtcaatcaactgtgccagttgctgggtgcaatgataaagtcccagcgccagcaacctaggggaggacaggccaaaaagaaaaagcctgagaagccacattttcccctggctgctgaagatgacatccggcaccacctcacccagactgaacgctccctctgcttgcaatcgatccagacggctttcaatcaaggcgcaggaactgcgtcgctttcatccagcgggaaggtcagttttcaggttgagtttatgctgccggttgctcatacagtgcgcctgattcgcgtgacttctacatccgccagtcagggtgcaagttaatttgacagtcaggtgaatggccgcgatggcgtgtggcctctgagtcacctattcaattagggcgatcacatgggggtcatacttaattcaggcaggaaccatgtgaccgaaattaaaaaaaaaaaaaaaaaaaa

SEQ ID NO: 30 - DNA, 34864 bp, Artificial Sequence
  pAd/PL-DEST vector; attR1 site: 512-636; attR2 site: 2092-2216
  misc_feature (34060)..(34060): n is a, c, g, or t
catcatcaataatataccttattttggattgaagccaatatgataatgagggggtggagtttgtgacgtggcgcggggcgtgggaacggggcgggtgacgtagtagtgtggcggaagtgtgatgttgcaagtgtggcggaacacatgtaagcgacggatgtggcaaaagtgacgtttttggtgtgcgccggtgtacacaggaagtgacaattttcgcgcggttttaggcggatgttgtagtaaatttgggcgtaaccgagtaagatttggccattttcgcgggaaaactgaataagaggaagtgaaatctgaataattttgtgttactcatagcgcgtaatatttgtctagggccgcggggactttgaccgtttacgtggagactcgcccaggtgtttttctcaggtgttttccgcgttccgggtcaaagttggcgttttattattatagtcagtcgaagcttggatccggtacctctagaattctcgagcggccgctagcgacatcgatcacaagtttgtacaaaaaagctgaacgagaaacgtaaaatgatataaatatcaatatattaaattagattttgcataaaaaacagactacataatactgtaaaacacaacatatccagtcactatggcggccgcattaggcaccccaggctttacactttatgcttccggctcgtataatgtgtggattttgagttaggatccggcgagattttcaggagctaaggaagctaaaatggagaaaaaaatcactggatataccaccgttgatatatcccaatggcatcgtaaagaacattttgaggcatttcagtcagttgctcaatgtacctataaccagaccgttcagctggatattacggcctttttaaagaccgtaaagaaaaataagcacaagttttatccggcctttattcacattcttgcccgcctgatgaatgctcatccggaattccgtatggcaatgaaagacggtgagctggtgatatgggatagtgttcacccttgttacaccgttttccatgagcaaactgaaacgttttcatcgctctggagtgaataccacgacgatttccggcagtttctacacatatattcgcaagatgtggcgtgttacggtgaaaacctggcctatttccctaaagggtttattgagaatatgtttttcgtctcagccaatccctgggtgagtttcaccagttttgatttaaacgtggccaatatggacaatttcttcgcccccgttttcaccatgggcaaatattatacgcaaggcgacaaggtgctgatgccgctggcgattcaggttcatcatgccgtctgtgatggcttccatgtcggcagaatgcttaatgaattacaacagtactgcgatgagtggcagggcggggcgtaaacgcgtggatccggcttactaaaaaccagataacagtatgcgtatttgcgcgctgatttttgcggtataagaatatatactgatatgtatacccgaagtatgtcaaaaagaggtgtgctatgaagcagcgtattacagtgacagttgacagcgacagctatcagttgctcaaggcatatatgatgtcaatatctccggtctggtaagcacaaccatgcagaatgaagcccgtcgtctgcgtgccgaacgctggaaagcggaaaatcaggaagggatggctgaggtcgcccggtttattgaaatgaacggctcttttgctgacgagaacaggggctggtgaaatgcagtttaaggtttacacctataaaagagagagccgttatcgtctgtttgtggatgtacagagtgatattattgacacgcccgggcgacggatggtgatccccctggccagtgcacgtctgctgtcagataaagtctcccgtgaactttacccggtggtgcatatcggggatgaaagctggcgcatgatgaccaccgatatggccagtgtgccggtctccgttatcggggaagaagtggctgatctcagccaccgcgaaaatgacatcaaaaacgccattaacctgatgttctggggaatataaatgtcaggctcccttatacacagccagtctgcaggtcgaccatagtgactggatatgttgtgttttacagtattatgtagtctgttttttatgcaaaatctaatttaatatattgatatttatatcattttacgtttctcgttcagctttcttgtacaaagtggtgatcgattcgacagatcactgaaatgtgtgggcgtggcttaagggtgggaaagaatatataaggtgggggtcttatgtagttttgtatctgttttgcagcagccgccgccgccatgagcaccaactcgtttgatggaagcattgtgagctcatatttgacaacgcgcatgcccccatgggccggggtgcgtcagaatgtgatgggctccagcattgatggtcgccccgtcctgcccgcaaactctactaccttgacctacgagaccgtgtctggaacgccgttggagactgcagcctccgccgccgcttcagccgctgcagccaccgcccgcgggattgtgactgactttgctttcctgagcccgcttgcaagcagtgcagcttcccgttcatccgcccgcgatgacaagttgacggctcttttggcacaattggattctttgacccgggaacttaatgtcgtttctcagcagctgttggatctgcgccagcaggtttctgccctgaaggcttcctcccctcccaatgcggtttaaaacataaataaaaaaccagactctgtttggatttggatcaagcaagtgtcttgctgtctttatttaggggttttgcgcgcgcggtaggcccgggaccagcggtctcggtcgttgagggtcctgtgtattttttccaggacgtggtaaaggtgactctggatgttcagatacatgggcataagcccgtctctggggtggaggtagcaccactgcagagcttcatgctgcggggtggtgttgtagatgatccagtcgtagcaggagcgctgggcgtggtgcctaaaaatgtctttcagtagcaagctgattgccaggggcaggcccttggtgtaagtgtttacaaagcggttaagctgggatgggtgcatacgtggggatatgagatgcatcttggactgtatttttaggttggctatgttcccagccatatccctccggggattcatgttgtgcagaaccaccagcacagtgtatccggtgcacttgggaaatttgtcatgtagcttagaaggaaatgcgtggaagaacttggagacgcccttgtgacctccaagattttccatgcattcgtccataatgatggcaatgggcccacgggcggcggcctgggcgaagatatttctgggatcactaacgtcatagttgtgttccaggatgagatcgtcataggccatttttacaaagcgcgggcggagggtgccagactgcggtataatggttccatccggcccaggggcgtagttaccctcacagatttgcatttcccacgctttgagttcagatggggggatcatgtctacctgcggggcgatgaagaaaacggtttccggggtaggggagatcagctgggaagaaagcaggttcctgagcagctgcgacttaccgcagccggtgggcccgtaaatcacacctattaccgggtgcaactggtagttaagagagctgcagctgccgtcatccctgagcaggggggccacttcgttaagcatgtccctgactcgcatgttttccctgaccaaatccgccagaaggcgctcgccgcccagcgatagcagttcttgcaaggaagcaaagtttttcaacggtttgagaccgtccgccgtaggcatgcttttgagcgtttgaccaagcagttccaggcggtcccacagctcggtcacctgctctacggcatctcgatccagcatatctcctcgtttcgcgggttggggcggctttcgctgtacggcagtagtcggtgctcgtccagacgggccagggtcatgtctttccacgggcgcagggtcctcgtcagcgtagtctgggtcacggtgaaggggtgcgctccgggctgcgcgctggccagggtgcgcttgaggctggtcctgctggtgctgaagcgctgccggtcttcgccctgcgcgtcggccaggtagcatttgaccatggtgtcatagtccagcccctccgcggcgtggcccttggcgcgcagcttgcccttggaggaggcgccgcacgaggggcagtgcagacttttgagggcgtagagcttgggcgcgagaaataccgattccggggagtaggcatccgcgccgcaggccccgcagacggtctcgcattccacgagccaggtgagctctggccgttcggggtcaaaaaccaggtttcccccatgctttttgatgcgtttcttacctctggtttccatgagccggtgtccacgctcggtgacgaaaaggctgtccgtgtccccgtatacagacttgagaggcctgtcctcgagcggtgttccgcggtcctcctcgtatagaaactcggaccactctgagacaaaggctcgcgtccaggccagcacgaaggaggctaagtgggaggggtagcggtcgttgtccactagggggtccactcgctccagggtgtgaagacacatgtcgccctcttcggcatcaaggaaggtgattggtttgtaggtgtaggccacgtgaccgggtgttcctgaaggggggctataaaagggggtgggggcgcgttcgtcctcactctcttccgcatcgctgtctgcgagggccagctgttggggtgagtactccctctgaaaagcgggcatgacttctgcgctaagattgtcagtttccaaaaacgaggaggatttgatattcacctggcccgcggtgatgcctttgagggtggccgcatccatctggtcagaaaagacaatctttttgttgtcaagcttggtggcaaacgacccgtagagggcgttggacagcaacttggcgatggagcgcagggtttggtttttgtcgcgatcggcgcgctccttggccgcgatgtttagctgcacgtattcgcgcgcaacgcaccgccattcgggaaagacggtggtgcgctcgtcgggcaccaggtgcacgcgccaaccgcggttgtgcagggtgacaaggtcaacgctggtggctacctctccgcgtaggcgctcgttggtccagcagaggcggccgcccttgcgcgagcagaatggcggtagggggtctagctgcgtctcgtccggggggtctgcgtccacggtaaagaccccgggcagcaggcgcgcgtcgaagtagtctatcttgcatccttgcaagtctagcgcctgctgccatgcgcgggcggcaagcgcgcgctcgtatgggttgagtgggggaccccatggcatggggtgggtgagcgcggaggcgtacatgccgcaaatgtcgtaaacgtagaggggctctctgagtattccaagatatgtagggtagcatcttccaccgcggatgctggcgcgcacgtaatcgtatagttcgtgcgagggagcgaggaggtcgggaccgaggttgctacgggcgggctgctctgctcggaagactatctgcctgaagatggcatgtgagttggatgatatggttggacgctggaagacgttgaagctggcgtctgtgagacctaccgcgtcacgcacgaaggaggcgtaggagtcgcgcagcttgttgaccagctcggcggtgacctgcacgtctagggcgcagtagtccagggtttccttgatgatgtcatacttatcctgtcccttttttttccacagctcgcggttgaggacaaactcttcgcggtctttccagtactcttggatcggaaacccgtcggcctccgaacggtaagagcctagcatgtagaactggttgacggcctggtaggcgcagcatcccttttctacgggtagcgcgtatgcctgcgcggccttccggagcgaggtgtgggtgagcgcaaaggtgtccctgaccatgactttgaggtactggtatttgaagtcagtgtcgtcgcatccgccctgctcccagagcaaaaagtccgtgcgctttttggaacgcggatttggcagggcgaaggtgacatcgttgaagagtatctttcccgcgcgaggcataaagttgcgtgtgatgcggaagggtcccggcacctcggaacggttgttaattacctgggcggcgagcacgatctcgtcaaagccgttgatgttgtggcccacaatgtaaagttccaagaagcgcgggatgcccttgatggaaggcaattttttaagttcctcgtaggtgagctcttcaggggagctgagcccgtgctctgaaagggcccagtctgcaagatgagggttggaagcgacgaatgagctccacaggtcacgggccattagcatttgcaggtggtcgcgaaaggtcctaaactggcgacctatggccattttttctggggtgatgcagtagaaggtaagcgggtcttgttcccagcggtcccatccaaggttcgcggctaggtctcgcgcggcagtcactagaggctcatctccgccgaacttcatgaccagcatgaagggcacgagctgcttcccaaaggcccccatccaagtataggtctctacatcgtaggtgacaaagagacgctcggtgcgaggatgcgagccgatcgggaagaactggatctcccgccaccaattggaggagtggctattgatgtggtgaaagtagaagtccctgcgacgggccgaacactcgtgctggcttttgtaaaaacgtgcgcagtactggcagcggtgcacgggctgtacatcctgcacgaggttgacctgacgaccgcgcacaaggaagcagagtgggaatttgagcccctcgcctggcgggtttggctggtggtcttctacttcggctgcttgtccttgaccgtctggctgctcgaggggagttacggtggatcggaccaccacgccgcgcgagcccaaagtccagatgtccgcgcgcggcggtcggagcttgatgacaacatcgcgcagatgggagctgtccatggtctggagctcccgcggcgtcaggtcaggcgggagctcctgcaggtttacctcgcatagacgggtcagggcgcgggctagatccaggtgatacctaatttccaggggctggttggtggcggcgtcgatggcttgcaagaggccgcatccccgcggcgcgactacggtaccgcgcggcgggcggtgggccgcgggggtgtccttggatgatgcatctaaaagcggtgacgcgggcgagcccccggaggtagggggggctccggacccgccgggagagggggcaggggcacgtcggcgccgcgcgcgggcaggagctggtgctgcgcgcgtaggttgctggcgaacgcgacgacgcggcggttgatctcctgaatctggcgcctctgcgtgaagacgacgggcccggtgagcttgagcctgaaagagagttcgacagaatcaatttcggtgtcgttgacggcggcctggcgcaaaatctcctgcacgtctcctgagttgtcttgataggcgatctcggccatgaactgctcgatctcttcctcctggagatctccgcgtccggctcgctccacggtggcggcgaggtcgttggaaatgcgggccatgagctgcgagaaggcgttgaggcctccctcgttccagacgcggctgtagaccacgcccccttcggcatcgcgggcgcgcatgaccacctgcgcgagattgagctccacgtgccgggcgaagacggcgtagtttcgcaggcgctgaaagaggtagttgagggtggtggcggtgtgttctgccacgaagaagtacataacccagcgtcgcaacgtggattcgttgatatcccccaaggcctcaaggcgctccatggcctcgtagaagtccacggcgaagttgaaaaactgggagttgcgcgccgacacggttaactcctcctccagaagacggatgagctcggcgacagtgtcgcgcacctcgcgctcaaaggctacaggggcctcttcttcttcttcaatctcctcttccataagggcctccccttcttcttcttctggcggcggtgggggaggggggacacggcggcgacgacggcgcaccgggaggcggtcgacaaagcgctcgatcatctccccgcggcgacggcgcatggtctcggtgacggcgcggccgttctcgcgggggcgcagttggaagacgccgcccgtcatgtcccggttatgggttggcggggggctgccatgcggcagggatacggcgctaacgatgcatctcaacaattgttgtgtaggtactccgccgccgagggacctgagcgagtccgcatcgaccggatcggaaaacctctcgagaaaggcgtctaaccagtcacagtcgcaaggtaggctgagcaccgtggcgggcggcagcgggcggcggtcggggttgtttctggcggaggtgctgctgatgatgtaattaaagtaggcggtcttgagacggcggatggtcgacagaagcaccatgtccttgggtccggcctgctgaatgcgcaggcggtcggccatgccccaggcttcgttttgacatcggcgcaggtctttgtagtagtcttgcatgagcctttctaccggcacttcttcttctccttcctcttgtcctgcatctcttgcatctatcgctgcggcggcggcggagtttggccgtaggtggcgccctcttcctcccatgcgtgtgaccccgaagcccctcatcggctgaagcagggctaggtcggcgacaacgcgctcggctaatatggcctgctgcacctgcgtgagggtagactggaagtcatccatgtccacaaagcggtggtatgcgcccgtgttgatggtgtaagtgcagttggccataacggaccagttaacggtctggtgacccggctgcgagagctcggtgtacctgagacgcgagtaagccctcgagtcaaatacgtagtcgttgcaagtccgcaccaggtactggtatcccaccaaaaagtgcggcggcggctggcggtagaggggccagcgtagggtggccggggctccgggggcgagatcttccaacataaggcgatgatatccgtagatgtacctggacatccaggtgatgccggcggcggtggtggaggcgcgcggaaagtcgcggacgcggttccagatgttgcgcagcggcaaaaagtgctccatggtcgggacgctctggccggtcaggcgcgcgcaatcgttgacgctctagaccgtgcaaaaggagagcctgtaagcgggcactcttccgtggtctggtggataaattcgcaagggtatcatggcggacgaccggggttcgagccccgtatccggccgtccgccgtgatccatgcggttaccgcccgcgtgtcgaacccaggtgtgcgacgtcagacaacgggggagtgctccttttggcttccttccaggcgcggcggctgctgcgctagcttttttggccactggccgcgcgcagcgtaagcggttaggctggaaagcgaaagcattaagtggctcgctccctgtagccggagggttattttccaagggttgagtcgcgggacccccggttcgagtctcggaccggccggactgcggcgaacgggggtttgcctccccgtcatgcaagaccccgcttgcaaattcctccggaaacagggacgagccccttttttgcttttcccagatgcatccggtgctgcggcagatgcgcccccctcctcagcagcggcaagagcaagagcagcggcagacatgcagggcaccctcccctcctcctaccgcgtcaggaggggcgacatccgcggttgacgcggcagcagatggtgattacgaacccccgcggcgccgggcccggcactacctggacttggaggagggcgagggcctggcgcggctaggagcgccctctcctgagcggtacccaagggtgcagctgaagcgtgatacgcgtgaggcgtacgtgccgcggcagaacctgtttcgcgaccgcgagggagaggagcccgaggagatgcgggatcgaaagttccacgcagggcgcgagctgcggcatggcctgaatcgcgagcggttgctgcgcgaggaggactttgagcccgacgcgcgaaccgggattagtcccgcgcgcgcacacgtggcggccgccgacctggtaaccgcatacgagcagacggtgaaccaggagattaactttcaaaaaagctttaacaaccacgtgcgtacgcttgtggcgcgcgaggaggtggctataggactgatgcatctgtgggactttgtaagcgcgctggagcaaaacccaaatagcaagccgctcatggcgcagctgttccttatagtgcagcacagcagggacaacgaggcattcagggatgcgctgctaaacatagtagagcccgagggccgctggctgctcgatttgataaacatcctgcagagcatagtggtgcaggagcgcagcttgagcctggctgacaaggtggccgccatcaactattccatgcttagcctgggcaagttttacgcccgcaagatataccataccccttacgttcccatagacaaggaggtaaagatcgaggggttctacatgcgcatggcgctgaaggtgcttaccttgagcgacgacctgggcgtttatcgcaacgagcgcatccacaaggccgtgagcgtgagccggcggcgcgagctcagcgaccgcgagctgatgcacagcctgcaaagggccctggctggcacgggcagcggcgatagagaggccgagtcctactttgacgcgggcgctgacctgcgctgggccccaagccgacgcgccctggaggcagctggggccggacctgggctggcggtggcacccgcgcgcgctggcaacgtcggcggcgtggaggaatatgacgaggacgatgagtacgagccagaggacggcgagtactaagcggtgatgtttctgatcagatgatgcaagacgcaacggacccggcggtgcgggcggcgctgcagagccagccgtccggccttaactccacggacgactggcgccaggtcatggaccgcatcatgtcgctgactgcgcgcaatcctgacgcgttccggcagcagccgcaggccaaccggctctccgcaattctggaagcggtggtcccggcgcgcgcaaaccccacgcacgagaaggtgctggcgatcgtaaacgcgctggccgaaaacagggccatccggcccgacgaggccggcctggtctacgacgcgctgcttcagcgcgtggctcgttacaacagcggcaacgtgcagaccaacctggaccggctggtgggggatgtgcgcgaggccgtggcgcagcgtgagcgcgcgcagcagcagggcaacctgggctccatggttgcactaaacgccttcctgagtacacagcccgccaacgtgccgcggggacaggaggactacaccaactttgtgagcgcactgcggctaatggtgactgagacaccgcaaagtgaggtgtaccagtctgggccagactattttttccagaccagtagacaaggcctgcagaccgtaaacctgagccaggctttcaaaaacttgcaggggctgtggggggtgcgggctcccacaggcgaccgcgcgaccgtgtctagcttgctgacgcccaactcgcgcctgttgctgctgctaatagcgcccttcacggacagtggcagcgtgtcccgggacacatacctaggtcacttgctgacactgtaccgcgaggccataggtcaggcgcatgtggacgagcatactttccaggagattacaagtgtcagccgcgcgctggggcaggaggacacgggcagcctggaggcaaccctaaactacctgctgaccaaccggcggcagaagatcccctcgttgcacagtttaaacagcgaggaggagcgcattttgcgctacgtgcagcagagcgtgagccttaacctgatgcgcgacggggtaacgcccagcgtggcgctggacatgaccgcgcgcaacatggaaccgggcatgtatgcctcaaaccggccgtttatcaaccgcctaatggactacttgcatcgcgcggccgccgtgaaccccgagtatttcaccaatgccatcttgaacccgcactggctaccgccccctggtttctacaccgggggattcgaggtgcccgagggtaacgatggattcctctgggacgacatagacgacagcgtgttttccccgcaaccgcagaccctgctagagttgcaacagcgcgagcaggcagaggcggcgctgcgaaaggaaagcttccgcaggccaagcagcttgtccgatctaggcgctgcggccccgcggtcagatgctagtagcccatttccaagcttgatagggtctcttaccagcactcgcaccacccgcccgcgcctgctgggcgaggaggagtacctaaacaactcgctgctgcagccgcagcgcgaaaaaaacctgcctccggcatttcccaacaacgggatagagagcctagtggacaagatgagtagatggaagacgtacgcgcaggagcacagggacgtgccaggcccgcgcccgcccacccgtcgtcaaaggcacgaccgtcagcggggtctggtgtgggaggacgatgactcggcagacgacagcagcgtcctggatttgggagggagtggcaacccgtttgcgcaccttcgccccaggctggggagaatgttttaaaaaaaaaaaagcatgatgcaaaataaaaaactcaccaaggccatggcaccgagcgttggttttcttgtattccccttagtatgcggcgcgcggcgatgtatgaggaaggtcctcctccctcctacgagagtgtggtgagcgcggcgccagtggcggcggcgctgggttctcccttcgatgctcccctggacccgccgtttgtgcctccgcggtacctgcggcctaccggggggagaaacagcatccgttactctgagttggcacccctattcgacaccacccgtgtgtacctggtggacaacaagtcaacggatgtggcatccctgaactaccagaacgaccacagcaactttctgaccacggtcattcaaaacaatgactacagcccgggggaggcaagcacacagaccatcaatcttgacgaccggtcgcactggggcggcgacctgaaaaccatcctgcataccaacatgccaaatgtgaacgagttcatgtttaccaataagtttaaggcgcgggtgatggtgtcgcgcttgcctactaaggacaatcaggtggagctgaaatacgagtgggtggagttcacgctgcccgagggcaactactccgagaccatgaccatagaccttatgaacaacgcgatcgtggagcactacttgaaagtgggcagacagaacggggttctggaaagcgacatcggggtaaagtttgacacccgcaacttcagactggggtttgaccccgtcactggtcttgtcatgcctggggtatatacaaacgaagccttccatccagacatcattttgctgccaggatgcggggtggacttcacccacagccgcctgagcaacttgttgggcatccgcaagcggcaacccttccaggagggctttaggatcacctacgatgatctggagggtggtaacattcccgcactgttggatgtggacgcctaccaggcgagcttgaaagatgacaccgaacagggcgggggtggcgcaggcggcagcaacagcagtggcagcggcgcggaagagaactccaacgcggcagccgcggcaatgcagccggtggaggacatgaacgatcatgccattcgcggcgacacctttgccacacgggctgaggagaagcgcgctgaggccgaagcagcggccgaagctgccgcccccgctgcgcaacccgaggtcgagaagcctcagaagaaaccggtgatcaaacccctgacagaggacagcaagaaacgcagttacaacctaataagcaatgacagcaccttcacccagtaccgcagctggtaccttgcatacaactacggcgaccctcagaccggaatccgctcatggaccctgctttgcactcctgacgtaacctgcggctcggagcaggtctactggtcgttgccagacatgatgcaagaccccgtgaccttccgctccacgcgccagatcagcaactttccggtggtgggcgccgagctgttgcccgtgcactccaagagcttctacaacgaccaggccgtctactcccaactcatccgccagtttacctctctgacccacgtgttcaatcgctttcccgagaaccagattttggcgcgcccgccagcccccaccatcaccaccgtcagtgaaaacgttcctgctctcacagatcacgggacgctaccgctgcgcaacagcatcggaggagtccagcgagtgaccattactgacgccagacgccgcacctgcccctacgtttacaaggccctgggcatagtctcgccgcgcgtcctatcgagccgcactttttgagcaagcatgtccatccttatatcgcccagcaataacacaggctggggcctgcgcttcccaagcaagatgtttggcggggccaagaagcgctccgaccaacacccagtgcgcgtgcgcgggcactaccgcgcgccctggggcgcgcacaaacgcggccgcactgggcgcaccaccgtcgatgacgccatcgacgcggtggtggaggaggcgcgcaactacacgcccacgccgccaccagtgtccacagtggacgcggccattcagaccgtggtgcgcggagcccggcgctatgctaaaatgaagagacggcggaggcgcgtagcacgtcgccaccgccgccgacccggcactgccgcccaacgcgcggcggcggccctgcttaaccgcgcacgtcgcaccggccgacgggcggccatgcgggccgctcgaaggctggccgcgggtattgtcactgtgccccccaggtccaggcgacgagcggccgccgcagcagccgcggccattagtgctatgactcagggtcgcaggggcaacgtgtattgggtgcgcgactcggttagcggcctgcgcgtgcccgtgcgcacccgccccccgcgcaactagattgcaagaaaaaactacttagactcgtactgttgtatgtatccagcggcggcggcgcgcaacgaagctatgtccaagcgcaaaatcaaagaagagatgctccaggtcatcgcgccggagatctatggccccccgaagaaggaagagcaggattacaagccccgaaagctaaagcgggtcaaaaagaaaaagaaagatgatgatgatgaacttgacgacgaggtggaactgctgcacgctaccgcgcccaggcgacgggtacagtggaaaggtcgacgcgtaaaacgtgttttgcgacccggcaccaccgtagtctttacgcccggtgagcgctccacccgcacctacaagcgcgtgtatgatgaggtgtacggcgacgaggacctgcttgagcaggccaacgagcgcctcggggagtttgcctacggaaagcggcataaggacatgctggcgttgccgctggacgagggcaacccaacacctagcctaaagcccgtaacactgcagcaggtgctgcccgcgcttgcaccgtccgaagaaaagcgcggcctaaagcgcgagtctggtgacttggcacccaccgtgcagctgatggtacccaagcgccagcgactggaagatgtcttggaaaaaatgaccgtggaacctgggctggagcccgaggtccgcgtgcggccaatcaagcaggtggcgccgggactgggcgtgcagaccgtggacgttcagatacccactaccagtagcaccagtattgccaccgccacagagggcatggagacacaaacgtccccggttgcctcagcggtggcggatgccgcggtgcaggcggtcgctgcggccgcgtccaagacctctacggaggtgcaaacggacccgtggatgtttcgcgtttcagccccccggcgcccgcgcggttcgaggaagtacggcgccgccagcgcgctactgcccgaatatgccctacatccttccattgcgcctacccccggctatcgtggctacacctaccgccccagaagacgagcaactacccgacgccgaaccaccactggaacccgccgccgccgtcgccgtcgccagcccgtgctggccccgatttccgtgcgcagggtggctcgcgaaggaggcaggaccctggtgctgccaacagcgcgctaccaccccagcatcgtttaaaagccggtctttgtggttcttgcagatatggccctcacctgccgcctccgtttcccggtgccgggattccgaggaagaatgcaccgtaggaggggcatggccggccacggcctgacgggcggcatgcgtcgtgcgcaccaccggcggcggcgcgcgtcgcaccgtcgcatgcgcggcggtatcctgcccctccttattccactgatcgccgcggcgattggcgccgtgcccggaattgcatccgtggccttgcaggcgcagagacactgattaaaaacaagttgcatgtggaaaaatcaaaataaaaagtctggactctcacgctcgcttggtcctgtaactattttgtagaatggaagacatcaactttgcgtctctggccccgcgacacggctcgcgcccgttcatgggaaactggcaagatatcggcaccagcaatatgagcggtggcgccttcagctggggctcgctgtggagcggcattaaaaatttcggttccaccgttaagaactatggcagcaaggcctggaacagcagcacaggccagatgctgagggataagttgaaagagcaaaatttccaacaaaaggtggtagatggcctggcctctggcattagcggggtggtggacctggccaaccaggcagtgcaaaataagattaacagtaagcttgatccccgccctcccgtagaggagcctccaccggccgtggagacagtgtctccagaggggcgtggcgaaaagcgtccgcgccccgacagggaagaaactctggtgacgcaaatagacgagcctccctcgtacgaggaggcactaaagcaaggcctgcccaccacccgtcccatcgcgcccatggctaccggagtgctgggccagcacacacccgtaacgctggacctgcctccccccgccgacacccagcagaaacctgtgctgccaggcccgaccgccgttgttgtaacccgtcctagccgcgcgtccctgcgccgcgccgccagcggtccgcgatcgttgcggcccgtagccagtggcaactggcaaagcacactgaacagcatcgtgggtctgggggtgcaatccctgaagcgccgacgatgcttctgaatagctaacgtgtcgtatgtgtgtcatgtatgcgtccatgtcgccgccagaggagctgctgagccgccgcgcgcccgctttccaagatggctaccccttcgatgatgccgcagtggtcttacatgcacatctcgggccaggacgcctcggagtacctgagccccgggctggtgcagtttgcccgcgccaccgagacgtacttcagcctgaataacaagtttagaaaccccacggtggcgcctacgcacgacgtgaccacagaccggtcccagcgtttgacgctgcggttcatccctgtggaccgtgaggatactgcgtactcgtacaaggcgcggttcaccctagctgtgggtgataaccgtgtgctggacatggcttccacgtactttgacatccgcggcgtgctggacaggggccctacttttaagccctactctggcactgcctacaacgccctggctcccaagggtgccccaaatccttgcgaatgggatgaagctgctactgctcttgaaataaacctagaagaagaggacgatgacaacgaagacgaagtagacgagcaagctgagcagcaaaaaactcacgtatttgggcaggcgccttattctggtataaatattacaaaggagggtattcaaataggtgtcgaaggtcaaacacctaaatatgccgataaaacatttcaacctgaacctcaaataggagaatctcagtggtacgaaactgaaattaatcatgcagctgggagagtccttaaaaagactaccccaatgaaaccatgttacggttcatatgcaaaacccacaaatgaaaatggagggcaaggcattcttgtaaagcaacaaaatggaaagctagaaagtcaagtggaaatgcaatttttctcaactactgaggcgaccgcaggcaatggtgataacttgactcctaaagtggtattgtacagtgaagatgtagatatagaaaccccagacactcatatttcttacatgcccactattaaggaaggtaactcacgagaactaatgggccaacaatctatgcccaacaggcctaattacattgcttttagggacaattttattggtctaatgtattacaacagcacgggtaatatgggtgttctggcgggccaagcatcgcagttgaatgctgttgtagatttgcaagacagaaacacagagctttcataccagcttttgcttgattccattggtgatagaaccaggtacttttctatgtggaatcaggctgttgacagctatgatccagatgttagaattattgaaaatcatggaactgaagatgaacttccaaattactgctttccactgggaggtgtgattaatacagagactcttaccaaggtaaaacctaaaacaggtcaggaaaatggatgggaaaaagatgctacagaattttcagataaaaatgaaataagagttggaaataattttgccatggaaatcaatctaaatgccaacctgtggagaaatttcctgtactccaacatagcgctgtatttgcccgacaagctaaagtacagtccttccaacgtaaaaatttctgataacccaaacacctacgactacatgaacaagcgagtggtggctcccgggttagtggactgctacattaaccttggagcacgctggtcccttgactatatggacaacgtcaacccatttaaccaccaccgcaatgctggcctgcgctaccgctcaatgttgctgggcaatggtcgctatgtgcccttccacatccaggtgcctcagaagttctttgccattaaaaacctccttctcctgccgggctcatacacctacgagtggaacttcaggaaggatgttaacatggttctgcagagctccctaggaaatgacctaagggttgacggagccagcattaagtttgatagcatttgcctttacgccaccttcttccccatggcccacaacaccgcctccacgcttgaggccatgcttagaaacgacaccaacgaccagtcctttaacgactatctctccgccgccaacatgctctaccctatacccgccaacgctaccaacgtgcccatatccatcccctcccgcaactgggcggctttccgcggctgggccttcacgcgccttaagactaaggaaaccccatcactgggctcgggctacgacccttattacacctactctggctctataccctacctagatggaaccttttacctcaaccacacctttaagaaggtggccattacctttgactcttctgtcagctggcctggcaatgaccgcctgcttacccccaacgagtttgaaattaagcgctcagttgacggggagggttacaacgttgcccagtgtaacatgaccaaagactggttcctggtacaaatgctagctaactacaacattggctaccagggcttctatatcccagagagctacaaggaccgcatgtactccttctttagaaacttccagcccatgagccgtcaggtggtggatgatactaaatacaaggactaccaacaggtgggcatcctacaccaacacaacaactctggatttgttggctaccttgcccccaccatgcgcgaaggacaggcctaccctgctaacttcccctatccgcttataggcaagaccgcagttgacagcattacccagaaaaagtttctttgcgatcgcaccctttggcgcatcccattctccagtaactttatgtccatgggcgcactcacagacctgggccaaaaccttctctacgccaactccgcccacgcgctagacatgacttttgaggtggatcccatggacgagcccacccttctttatgttttgtttgaagtctttgacgtggtccgtgtgcaccggccgcaccgcggcgtcatcgaaaccgtgtacctgcgcacgcccttctcggccggcaacgccacaacataaagaagcaagcaacatcaacaacagctgccgccatgggctccagtgagcaggaactgaaagccattgtcaaagatcttggttgtgggccatattttttgggcacctatgacaagcgctttccaggctttgtttctccacacaagctcgcctgcgccatagtcaatacggccggtcgcgagactgggggcgtacactggatggcctttgcctggaacccgcactcaaaaacatgctacctctttgagccctttggcttttctgaccagcgactcaagcaggtttaccagtttgagtacgagtcactcctgcgccgtagcgccattgcttcttcccccgaccgctgtataacgctggaaaagtccacccaaagcgtacaggggcccaactcggccgcctgtggactattctgctgcatgtttctccacgcctttgccaactggccccaaactcccatggatcacaaccccaccatgaaccttattaccggggtacccaactccatgctcaacagtccccaggtacagcccaccctgcgtcgcaaccaggaacagctctacagcttcctggagcgccactcgccctacttccgcagccacagtgcgcagattaggagcgccacttctttttgtcacttgaaaaacatgtaaaaataatgtactagagacactttcaataaaggcaaatgcttttatttgtacactctcgggtgattatttacccccacccttgccgtctgcgccgtttaaaaatcaaaggggttctgccgcgcatcgctatgcgccactggcagggacacgttgcgatactggtgtttagtgctccacttaaactcaggcacaaccatccgcggcagctcggtgaagttttcactccacaggctgcgcaccatcaccaacgcgtttagcaggtcgggcgccgatatcttgaagtcgcagttggggcctccgccctgcgcgcgcgagttgcgatacacagggttgcagcactggaacactatcagcgccgggtggtgcacgctggccagcacgctcttgtcggagatcagatccgcgtccaggtcctccgcgttgctcagggcgaacggagtcaactttggtagctgccttcccaaaaagggcgcgtgcccaggctttgagttgcactcgcaccgtagtggcatcaaaaggtgaccgtgcccggtctgggcgttaggatacagcgcctgcataaaagccttgatctgcttaaaagccacctgagcctttgcgccttcagagaagaacatgccgcaagacttgccggaaaactgattggccggacaggccgcgtcgtgcacgcagcaccttgcgtcggtgttggagatctgcaccacatttcggccccaccggttcttcacgatcttggccttgctagactgctccttcagcgcgcgctgcccgttttcgctcgtcacatccatttcaatcacgtgctccttatttatcataatgcttccgtgtagacacttaagctcgccttcgatctcagcgcagcggtgcagccacaacgcgcagcccgtgggctcgtgatgcttgtaggtcacctctgcaaacgactgcaggtacgcctgcaggaatcgccccatcatcgtcacaaaggtcttgttgctggtgaaggtcagctgcaacccgcggtgctcctcgttcagccaggtcttgcatacggccgccagagcttccacttggtcaggcagtagtttgaagttcgcctttagatcgttatccacgtggtacttgtccatcagcgcgcgcgcagcctccatgcccttctcccacgcagacacgatcggcacactcagcgggttcatcaccgtaatttcactttccgcttcgctgggctcttcctcttcctcttgcgtccgcataccacgcgccactgggtcgtcttcattcagccgccgcactgtgcgcttacctcctttgccatgcttgattagcaccggtgggttgctgaaacccaccatttgtagcgccacatcttctctttcttcctcgctgtccacgattacctctggtgatggcgggcgctcgggcttgggagaagggcgcttctttttcttcttgggcgcaatggccaaatccgccgccgaggtcgatggccgcgggctgggtgtgcgcggcaccagcgcgtcttgtgatgagtcttcctcgtcctcggactcgatacgccgcctcatccgcttttttgggggcgcccggggaggcggcggcgacggggacggggacgacacgtcctccatggttgggggacgtcgcgccgcaccgcgtccgcgctcgggggtggtttcgcgctgctcctcttcccgactggccatttccttctcctataggcagaaaaagatcatggagtcagtcgagaagaaggacagcctaaccgccccctctgagttcgccaccaccgcctccaccgatgccgccaacgcgcctaccaccttccccgtcgaggcacccccgcttgaggaggaggaagtgattatcgagcaggacccaggttttgtaagcgaagacgacgaggaccgctcagtaccaacagaggataaaaagcaagaccaggacaacgcagaggcaaacgaggaacaagtcgggcggggggacgaaaggcatggcgactacctagatgtgggagacgacgtgctgttgaagcatctgcagcgccagtgcgccattatctgcgacgcgttgcaagagcgcagcgatgtgcccctcgccatagcggatgtcagccttgcctacgaacgccacctattctcaccgcgcgtaccccccaaacgccaagaaaacggcacatgcgagcccaacccgcgcctcaacttctaccccgtatttgccgtgccagaggtgcttgccacctatcacatctttttccaaaactgcaagatacccctatcctgccgtgccaaccgcagccgagcggacaagcagctggccttgcggcagggcgctgtcatacctgatatcgcctcgctcaacgaagtgccaaaaatctttgagggtcttggacgcgacgagaagcgcgcggcaaacgctctgcaacaggaaaacagcgaaaatgaaagtcactctggagtgttggtggaactcgagggtgacaacgcgcgcctagccgtactaaaacgcagcatcgaggtcacccactttgcctacccggcacttaacctaccccccaaggtcatgagcacagtcatgagtgagctgatcgtgcgccgtgcgcagcccctggagagggatgcaaatttgcaagaacaaacagaggagggcctacccgcagttggcgacgagcagctagcgcgctggcttcaaacgcgcgagcctgccgacttggaggagcgacgcaaactaatgatggccgcagtgctcgttaccgtggagcttgagtgcatgcagcggttctttgctgacccggagatgcagcgcaagctagaggaaacattgcactacacctttcgacagggctacgtacgccaggcctgcaagatctccaacgtggagctctgcaacctggtctcctaccttggaattttgcacgaaaaccgccttgggcaaaacgtgcttcattccacgctcaagggcgaggcgcgccgcgactacgtccgcgactgcgtttacttatttctatgctacacctggcagacggccatgggcgtttggcagcagtgcttggaggagtgcaacctcaaggagctgcagaaactgctaaagcaaaacttgaaggacctatggacggccttcaacgagcgctccgtggccgcgcacctggcggacatcattttccccgaacgcctgcttaaaaccctgcaacagggtctgccagacttcaccagtcaaagcatgttgcagaactttaggaactttatcctagagcgctcaggaatcttgcccgccacctgctgtgcacttcctagcgactttgtgcccattaagtaccgcgaatgccctccgccgctttggggccactgctaccttctgcagctagccaactaccttgcctaccactctgacataatggaagacgtgagcggtgacggtctactggagtgtcactgtcgctgcaacctatgcaccccgcaccgctccctggtttgcaattcgcagctgcttaacgaaagtcaaattatcggtacctttgagctgcagggtccctcgcctgacgaaaagtccgcggctccggggttgaaactcactccggggctgtggacgtcggcttaccttcgcaaatttgtacctgaggactaccacgcccacgagattaggttctacgaagaccaatcccgcccgccaaatgcggagcttaccgcctgcgtcattacccagggccacattcttggccaattgcaagccatcaacaaagcccgccaagagtttctgctacgaaagggacggggggtttacttggacccccagtccggcgaggagctcaacccaatccccccgccgccgcagccctatcagcagcagccgcgggcccttgcttcccaggatggcacccaaaaagaagctgcagctgccgccgccacccacggacgaggaggaatactgggacagtcaggcagaggaggttttggacgaggaggaggaggacatgatggaagactgggagagcctagacgaggaagcttccgaggtcgaagaggtgtcagacgaaacaccgtcaccctcggtcgcattcccctcgccggcgccccagaaatcggcaaccggttccagcatggctacaacctccgctcctcaggcgccgccggcactgcccgttcgccgacccaaccgtagatgggacaccactggaaccagggccggtaagtccaagcagccgccgccgttagcccaagagcaacaacagcgccaaggctaccgctcatggcgcgggcacaagaacgccatagttgcttgcttgcaagactgtgggggcaacatctccttcgcccgccgctttcttctctaccatcacggcgtggccttcccccgtaacatcctgcattactaccgtcatctctacagcccatactgcaccggcggcagcggcagcggcagcaacagcagcggccacacagaagcaaaggcgaccggatagcaagactctgacaaagcccaagaaatccacagcggcggcagcagcaggaggaggagcgctgcgtctggcgcccaacgaacccgtatcgacccgcgagcttagaaacaggatttttcccactctgtatgctatatttcaacagagcaggggccaagaacaagagctgaaaataaaaaacaggtctctgcgatccctcacccgcagctgcctgtatcacaaaagcgaagatcagcttcggcgcacgctggaagacgcggaggctctcttcagtaaatactgcgcgctgactcttaaggactagtttcgcgccctttctcaaatttaagcgcgaaaactacgtcatctccagcggccacacccggcgccagcacctgtcgtcagcgccattatgagcaaggaaattcccacgccctacatgtggagttaccagccacaaatgggacttgcggctggagctgcccaagactactcaacccgaataaactacatgagcgcgggaccccacatgatatcccgggtcaacggaatccgcgcccaccgaaaccgaattctcttggaacaggcggctattaccaccacacctcgtaataaccttaatccccgtagttggcccgctgccctggtgtaccaggaaagtcccgctcccaccactgtggtacttcccagagacgcccaggccgaagttcagatgactaactcaggggcgcagcttgcgggcggctttcgtcacagggtgcggtcgcccgggcagggtataactcacctgacaatcagagggcgaggtattcagctcaacgacgagtcggtgagctcctcgcttggtctccgtccggacgggacatttcagatcggcggcgccggccgtccttcattcacgcctcgtcaggcaatcctaactctgcagacctcgtcctctgagccgcgctctggaggcattggaactctgcaatttattgaggagtttgtgccatcggtctactttaaccccttctcgggacctcccggccactatccggatcaatttattcctaactttgacgcggtaaaggactcggcggacggctacgactgaatgttaagtggagaggcagagcaactgcgcctgaaacacctggtccactgtcgccgccacaagtgctttgcccgcgactccggtgagttttgctactttgaattgcccgaggatcatatcgagggcccggcgcacggcgtccggcttaccgcccagggagagcttgcccgtagcctgattcgggagtttacccagcgccccctgctagttgagcgggacaggggaccctgtgttctcactgtgatttgcaactgtcctaaccttggattacatcaagatctttgttgccatctctgtgctgagtataataaatacagaaattaaaatatactggggctcctatcgccatcctgtaaacgccaccgtcttcacccgcccaagcaaaccaaggcgaaccttacctggtacttttaacatctctccctctgtgatttacaacagtttcaacccagacggagtgagtctacgagagaacctctccgagctcagctactccatcagaaaaaacaccaccctccttacctgccgggaacgtacgagtgcgtcaccggccgctgcaccacacctaccgcctgaccgtaaaccagactttttccggacagacctcaataactctgtttaccagaacaggaggtgagcttagaaaacccttagggtattaggccaaaggcgcagctactgtggggtttatgaacaattcaagcaactctacgggctattctaattcaggtttctctagaaatggacggaattattacagagcagcgcctgctagaaagacgcagggcagcggccgagcaacagcgcatgaatcaagagctccaagacatggttaacttgcaccagtgcaaaaggggtatcttttgtctggtaaagcaggccaaagtcacctacgacagtaataccaccggacaccgccttagctacaagttgccaaccaagcgtcagaaattggtggtcatggtgggagaaaagcccattaccataactcagcactcggtagaaaccgaaggctgcattcactcaccttgtcaaggacctgaggatctctgcacccttattaagaccctgtgcggtctcaaagatcttattccctttaactaataaaaaaaaataataaagcatcacttacttaaaatcagttagcaaatttctgtccagtttattcagcagcacctccttgccctcctcccagctctggtattgcagcttcctcctggctgcaaactttctccacaatctaaatggaatgtcagtttcctcctgttcctgtccatccgcacccactatcttcatgttgttgcagatgaagcgcgcaagaccgtctgaagataccttcaaccccgtgtatccatatgacacggaaaccggtcctccaactgtgccttttcttactcctccctttgtatcccccaatgggtttcaagagagtccccctggggtactctctttgcgcctatccgaacctctagttacctccaatggcatgcttgcgctcaaaatgggcaacggcctctctctggacgaggccggcaaccttacctcccaaaatgtaaccactgtgagcccacctctcaaaaaaaccaagtcaaacataaacctggaaatatctgcacccctcacagttacctcagaagccctaactgtggctgccgccgcacctctaatggtcgcgggcaacacactcaccatgcaatcacaggccccgctaaccgtgcacgactccaaacttagcattgccacccaaggacccctcacagtgtcagaaggaaagctagccctgcaaacatcaggccccctcaccaccaccgatagcagtacccttactatcactgcctcaccccctctaactactgccactggtagcttgggcattgacttgaaagagcccatttatacacaaaatggaaaactaggactaaagtacggggctcctttgcatgtaacagacgacctaaacactttgaccgtagcaactggtccaggtgtgactattaataatacttccttgcaaactaaagttactggagccttgggttttgattcacaaggcaatatgcaacttaatgtagcaggaggactaaggattgattctcaaaacagacgccttatacttgatgttagttatccgtttgatgctcaaaaccaactaaatctaagactaggacagggccctctttttataaactcagcccacaacttggatattaactacaacaaaggcctttacttgtttacagcttcaaacaattccaaaaagcttgaggttaacctaagcactgccaaggggttgatgtttgacgctacagccatagccattaatgcaggagatgggcttgaatttggttcacctaatgcaccaaacacaaatcccctcaaaacaaaaattggccatggcctagaatttgattcaaacaaggctatggttcctaaactaggaactggccttagttttgacagcacaggtgccattacagtaggaaacaaaaataatgataagctaactttgtggaccacaccagctccatctcctaactgtagactaaatgcagagaaagatgctaaactcactttggtcttaacaaaatgtggcagtcaaatacttgctacagtttcagttttggctgttaaaggcagtttggctccaatatctggaacagttcaaagtgctcatcttattataagatttgacgaaaatggagtgctactaaacaattccttcctggacccagaatattggaactttagaaatggagatcttactgaaggcacagcctatacaaacgctgttggatttatgcctaacctatcagcttatccaaaatctcacggtaaaactgccaaaagtaacattgtcagtcaagtttacttaaacggagacaaaactaaacctgtaacactaaccattacactaaacggtacacaggaaacaggagacacaactccaagtgcatactctatgtcattttcatgggactggtctggccacaactacattaatgaaatatttgccacatcctcttacactttttcatacattgcccaagaataaagaatcgtttgtgttatgtttcaacgtgtttatttttcaattgcagaaaatttcgaatcatttttcattcagtagtatagccccaccaccacatagcttatacagatcaccgtaccttaatcaaactcacagaaccctagtattcaacctgccacctccctcccaacacacagagtacacagtcctttctccccggctggccttaaaaagcatcatatcatgggtaacagacatattcttaggtgttatattccacacggtttcctgtcgagccaaacgctcatcagtgatattaataaactccccgggcagctcacttaagttcatgtcgctgtccagctgctgagccacaggctgctgtccaacttgcggttgcttaacgggcggcgaaggagaagtccacgcctacatgggggtagagtcataatcgtgcatcaggatagggcggtggtgctgcagcagcgcgcgaataaactgctgccgccgccgctccgtcctgcaggaatacaacatggcagtggtctcctcagcgatgattcgcaccgcccgcagcataaggcgccttgtcctccgggcacagcagcgcaccctgatctcacttaaatcagcacagtaactgcagcacagcaccacaatattgttcaaaatcccacagtgcaaggcgctgtatccaaagctcatggcggggaccacagaacccacgtggccatcataccacaagcgcaggtagattaagtggcgacccctcataaacacgctggacataaacattacctcttttggcatgttgtaattcaccacctcccggtaccatataaacctctgattaaacatggcgccatccaccaccatcctaaaccagctggccaaaacctgcccgccggctatacactgcagggaaccgggactggaacaatgacagtggagagcccaggactcgtaaccatggatcatcatgctcgtcatgatatcaatgttggcacaacacaggcacacgtgcatacacttcctcaggattacaagctcctcccgcgttagaaccatatcccagggaacaacccattcctgaatcagcgtaaatcccacactgcagggaagacctcgcacgtaactcacgttgtgcattgtcaaagtgttacattcgggcagcagcggatgatcctccagtatggtagcgcgggtttctgtctcaaaaggaggtagacgatccctactgtacggagtgcgccgagacaaccgagatcgtgttggtcgtagtgtcatgccaaatggaacgccggacgtagtcatatttcctgaagcaaaaccaggtgcgggcgtgacaaacagatctgcgtctccggtctcgccgcttagatcgctctgtgtagtagttgtagtatatccactctctcaaagcatccaggcgccccctggcttcgggttctatgtaaactccttcatgcgccgctgccctgataacatccaccaccgcagaataagccacacccagccaacctacacattcgttctgcgagtcacacacgggaggagcgggaagagctggaagaaccatgtttttttttttattccaaaagattatccaaaacctcaaaatgaagatctattaagtgaacgcgctcccctccggtggcgtggtcaaactctacagccaaagaacagataatggcatttgtaagatgttgcacaatggcttccaaaaggcaaacggccctcacgtccaagtggacgtaaaggctaaacccttcagggtgaatctcctctataaacattccagcaccttcaaccatgcccaaataattctcatctcgccaccttctcaatatatctctaagcaaatcccgaatattaagtccggccattgtaaaaatctgctccagagcgccctccaccttcagcctcaagcagcgaatcatgattgcaaaaattcaggttcctcacagacctgtataagattcaaaagcggaacattaacaaaaataccgcgatcccgtaggtcccttcgcagggccagctgaacataatcgtgcaggtctgcacggaccagcgcggccacttccccgccaggaaccttgacaaaagaacccacactgattatgacacgcatactcggagctatgctaaccagcgtagccccgatgtaagctttgttgcatgggcggcgatataaaatgcaaggtgctgctcaaaaaatcaggcaaagcctcgcgcaaaaaagaaagcacatcgtagtcatgctcatgcagataaaggcaggtaagctccggaaccaccacagaaaaagacaccatttttctctcaaacatgtctgcgggtttctgcataaacacaaaataaaataacaaaaaaacatttaaacattagaagcctgtcttacaacaggaaaaacaacccttataagcataagacggactacggccatgccggcgtgaccgtaaaaaaactggtcaccgtgattaaaaagcaccaccgacagctcctcggtcatgtccggagtcataatgtaagactcggtaaacacatcaggttgattcacatcggtcagtgctaaaaagcgaccgaaatagcccgggggaatacatacccgcaggcgtagagacaacattacagcccccataggaggtataacaaaattaataggagagaaaaacacataaacacctgaaaaaccctcctgcctaggcaaaatagcaccctcccgctccagaacaacatacagcgcttccacagcggcagccataacagtcagccttaccagtaaaaaagaaaacctattaaaaaaacaccactcgacacggcaccagctcaatcagtcacagtgtaaaaaagggccaagtgcagagcgagtatatataggactaaaaaatgacgtaacggttaaagtccacaaaaaacacccagaaaaccgcacgcgaacctacgcccagaaacgaaagccaaaaaacccacaacttcctcaaatcgtcacttccgttttcccacgttacgtcacttcccattttaagaaaactacaattcccaacacatacaagttactccgccctaaaacctacgtcacccgccccgttcccacgccccgcgccacgtcacaaactccaccccctcattatcatattggcttcaatccaaaataaggtatattattgatgatgttaattaatttaaatccgcatgcgatatcgagctctcccgggaattcggatctgcgacgcgaggctggatggccttccccattatgattcttctcgcttccggcggcatcgggatgcccgcgttgcaggccatgctgtccaggcaggtagatgacgaccatcagggacagcttcacggccagcaaaaggccaggaaccgtaaaaaggccgcgttgctggcgtttttccataggctccgcccccctgacgagcatcacaaaaatcgacgctcaagtcagaggtggcgaaacccgacaggactataaagataccaggcgtttccccctggaagctccctcgtgcgctctcctgttccgaccctgccgcttaccggatacctgtccgcctttctcccttcgggaagcgtggcgctttctcaatgctcacgctgtaggtatctcagttcggtgtaggtcgttcgctccaagctgggctgtgtgcacgaaccccccgttcagcccgaccgctgcgccttatccggtaactatcgtcttgagtccaacccggtaagacacgacttatcgccactggcagcagccactggtaacaggattagcagagcgaggtatgtaggcggtgctacagagttcttgaagtggtggcctaactacggctacactagaaggacagtatttggtatctgcgctctgctgaagccagttaccttcggaaaaagagttggtagctcttgatccggcaaacaaaccaccgctggtagcggtggtttttttgtttgcaagcagcagattacgcgcagaaaaaaaggatctcaagaagatcctttgatcttttctacggggtctgacgctcagtggaacgaaaactcacgttaagggattttggtcatgagattatcaaaaaggatcttcacctagatccttttaaatcaatctaaagtatatatgagtaaacttggtctgacagttaccaatgcttaatcagtgaggcacctatctcagcgatctgtctatttcgttcatccatagttgcctgactccccgtcgtgtagataactacgatacgggagggcttaccatctggccccagtgctgcaatgataccgcgagacccacgctcaccggctccagatttatcagcaataaaccagccagccggaagggccgagcgcagaagtggtcctgcaactttatccgcctccatccagtctattaattgttgccgggaagctagagtaagtagttcgccagttaatagtttgcgcaacgttgttgccattgntgcaggcatcgtggtgtcacgctcgtcgtttggtatggcttcattcagctccggttcccaacgatcaaggcgagttacatgatcccccatgttgtgcaaaaaagcggttagctccttcggtcctccgatcgttgtcagaagtaagttggccgcagtgttatcactcatggttatggcagcactgcataattctcttactgtcatgccatccgtaagatgcttttctgtgactggtgagtactcaaccaagtcattctgagaatagtgtatgcggcgaccgagttgctcttgcccggcgtcaacacgggataataccgcgccacatagcagaactttaaaagtgctcatcattggaaaacgttcttcggggcgaaaactctcaaggatcttaccgctgttgagatccagttcgatgtaacccactcgtgcacccaactgatcttcagcatcttttactttcaccagcgtttctgggtgagcaaaaacaggaaggcaaaatgccgcaaaaaagggaataagggcgacacggaaatgttgaatactcatactcttcctttttcaatattattgaagcatttatcagggttattgtctcatgagcggatacatatttgaatgtatttagaaaaataaacaaataggggttccgcgcacatttccccgaaaagtgccacctgacgtctaagaaaccattattatcatgacattaacctataaaaataggcgtatcacgaggccctttcgtcttcaaggatccgaattcccgggagagctcgatatcgcatgcggatttaaattaattaa

SEQ ID NO: 31 - protein, 46 aa, Artificial Sequence
  PRRSV gp5a
MFKYVGEVLDRVLLLAIAFFVVYRAVLSCCARQRQQQQQLSYSVDL

SEQ ID NO: 32 - protein, 174 aa, Artificial Sequence
  VR2332 PRRSV M (matrix protein)
MGSSLDDFCHDSTAPQKVLLAFSITYTPVMIYALKVSRGRLLGLLHLLIFLNCAFTFGYMTFAHFQSTNKVALTMGAVVALLWGVYSAIETWKFITSRCRLCLLGRKYILAPAHHVESAARFHPIAANDNHAFVVRRPGSTTVNGTLVPGLKSLVLGGRKAVKQGVVNLVKYAK

SEQ ID NO: 33 - protein, 123 aa, Artificial Sequence
  VR2332 PRRSV N (nucleocapsid protein)
MPNNNGKQQKRKKGDGQPVNQLCQMLGKIIAQQNQSRGKGPGKKNKKKNPEKPHFPLATEDDVRHHFTPSERQLCLSSIQTAFNQGAGTCTLSDSGRISYTVEFSLPTHHTVRLIRVTASPSA

SEQ ID NO: 34 - protein, 256 aa, Artificial Sequence
  ABO40192.1 PRRSV gp2
MKWGLCKAFSTKLANFLWMLSRNFWCPLLISSYFWPFCLASQSQVGWWSSVSDWFAPRYSVRALPFTLSNYRRSYEAFLSQCQVDIPTWGTKHPLGMFWHHKVSTLIDEMVSRRMYRIMEKAGQAAWKQVVSEATLSRISSLDVVAHFQHLAAIEAETCKYLASRLPMLHNLRMTGSNVTIVYNSTLEQVVAIFPTPGSRPKLHDFQQWLIAVHSSIFSSVAASCTLFVVLWLRIPMLRTVFGFHWLGAIFLSNSQ

SEQ ID NO: 35 - protein, 256 aa, Artificial Sequence
  ACF93748.1 PRRSV gp2
MKWGLCKASLTKLANFLWMLSRNFWCPLLISSYFWPFCLASPSPVGWWSFASDWFAPRYSVRALPFTLSNYRRSYEAFLSQCQVDIPTWGFKHPLGMLWHHKVSTLIDEMVSRRMYRTMEKAGQAAWKQVVSEATLSRISGLDVVAHFQHLAAIEAETCKYLASRLPMLHNLRMTGSNVTIVYNSTSNQVFAIFPTPGSRPKRHDFQQWLIAVHSSIFSSVAASCTLFVVLWLRIPMLRSVFGFRWLGAIFLLNSR

SEQ ID NO: 36 - protein, 256 aa, Artificial Sequence
  AHA83141.1 PRRSV gp2
MKWGPYKAFLTKLANFLWMLSRSSWCPLLISLYFWPFCLASPSPVGWWSFASDWFAPRYSVRALPFTLSNYRRSYEAFLSQCQVDIPTWGTKHPLGMFWHHKVSTLIDEMVSRRMYRIMEKAGQAAWKQVVSEATLSRISSLDVVAHFQHLAAIEAETCKYLASRLPMLHNLRMTGSNVTIVYNSTLSQVFAIFPTPGSRPKLHDFQQWLIAVHSSIFSSVAASCTLFVVLWLRVPILHTVFGFRWLGAIFLSNSQ

SEQ ID NO: 37 - protein, 249 aa, Artificial Sequence
  CAA01838.1 Lelystad PRRSV gp2
MQWGHCGVKSASCSWTPSLSSLLVWLILPFSLPYCLGSPSQDGYWSFFSEWFAPRFSVRALPFTLPNYRRSYEGLLPNCRPDVPQFAVKHPLGMFWHMRVSHLIDEMVSRRIYQTMEHSGQAAWKQVVGEATLTKLSGLDIVTHFQHLAAVEADSCRFLSSRLVMLKNLAVGNVSLQYNTTLDRVELIFPTPGTRPKLTDFRQWLISVHASIFSSVASSVTLFIVLWLRIPALRYVFGFHWPTATHHSS

SEQ ID NO: 38 - protein, 256 aa, Artificial Sequence
  AAE74522.1 gp2
MQWGPCKAFLTRSVNFLWMLSRSSWCPLLISSYFWPFCLASPLPAGWWSFASDWFAPRYSVRALPFTLSNYRRSYEAFLSQCQVDIPAWGTRHPLGMLWHHKVSTLIDEMVSRRMYRIMEKAGQAAWKQVVSEATLSRISGLDVVAHFQHLAAIEAETCKYLASRLPMLHNLRITGSNVTIVHNSTLNQVFAIFPTPGSRPKLHDFQQWLIAVHSSISSSVAASCTLFVVLWLRMPMLRSVFGFRWLGAIFPSSSW

SEQ ID NO: 39 - protein, 249 aa, Artificial Sequence
  AAB54503.1 PRRSV gp2
  misc_feature (29)..(29): Xaa can be any naturally occurring amino acid
  misc_feature (93)..(93): Xaa can be any naturally occurring amino acid
  misc_feature (107)..(107): Xaa can be any naturally occurring amino acid
MQWGHCGVKSASCSWTPSLSSLLVWLILXFSLPYCLGSPSQDGYWSFFSEWFAPRFSVRALPFTLPNYRRSYEGLLPNCRPDVPQFAVKHPLXMFWHMRVSHLIDEXVSRRIYQTMEHSGQAAWKQVVGEATLTKLSGLDIVTHFQHLAAVEADSCRFLSSRLVMLKNLAVGNVSLQYNTTLDRVELIFPTPGTRPKLTDFRQWLISVHASIFSSVASSVTLFIVLWLRIPALRYVFGFHWPTATHHSS

SEQ ID NO: 40 - protein, 254 aa, Artificial Sequence
  AAE68461.1 PRRSV gp3
MVNSCTFLHIFLCCSFLYSLCCAVVAGSNTTYCFWFPLVRGNFSFELTVNYTVCPPCLTRQAAAEAYEPGRSLWCRIGYDRCGEDDHDELGFMVPSGLSSEGHLTSVYAWLAFLSFSYTAQFHPEIFGIGNVSRVYVDIEHQLICAEHDGQNTTLPRHDNISAVFQTYYQHQVDGGNWFHLEWLRPFFSSWLVLNVSWFLRRSPANHVSVRVLQTLRPTPPQRQALLSSKTSVALGIATRPLRRFAKSLSAVRR

SEQ ID NO: 41 - protein, 254 aa, Artificial Sequence
  AAQ51784.1 PRRSV gp3
MANSCTFLYIFLCCSFLYSFCCAVVAGSNATYCFWFPLVRGNFSFELTVNYTVCPPCLTRQAAAEAYEPGRSLWCRIGHDRCGEDDHDELGFVVPSGLSSEGHLTSAYAWLASLSFSYTAQFHPEIFGIGNVSRVYVDIKHQFICAVHDGQNTTLPHHDNISAVLQTYYQHQVDGGNWFHLEWVRPFFSSWLVLNVSWFLRRSPASHVSVRVFQTSRPTPPQRQALLSSKTSVALGIATRPLRRFAKSLSAARR

SEQ ID NO: 42 - protein, 254 aa, Artificial Sequence
  AAE74530.1 PRRSV gp3
MANSCTFLHILLCCSFLYSFCCVVVTDANATFCFWFPLVRGNFSFELMVNYTVCPPCLTRQAAAQIYEPNRSLWCRIGNDRCGEDDHDELGFTVPPGLSKEVHLTSVYAWLAFLSFSYTAQFHPEIFGIGNVSKVYVDINHQLICAVHDGQNTTLPRHDNISAVFQTYYQHQVDGGNWFHLEWLRPFFSSWLVLNVSWFLRRSPASHVSVRVFQTSRPTPPRQQISLSSRTSAALGMATRPLRRFAKSLSAARR

SEQ ID NO: 43 - protein, 265 aa, Artificial Sequence
  CAA01839.1 PRRSV gp3
MAHQCARFHFFLCGFICYLVHSALASNSSSTLCFWFPLAHGNTSFELTINYTICMPCSTSQAARQRLEPGRNMWCKIGHDRCEERDHDELLMSIPSGYGQLKLEGYYAWLAFLSFSYAAQFHPELFGIGNVSRVFVDKRHQFICAEHDGHNSTVSTGHNISALYAAYYHHQIDGGNWFHLEWLRPLFSSWLVLNISWFLRRSPVSPVSRRIYQILRPTRPRLPVSWSFRTSIVSDLTGSQQRKRKFPSESRPNVVKPSVLPSTSR

SEQ ID NO: 44 - protein, 265 aa, Artificial Sequence
  ABH73414.1 PRRSV gp3
MAHQCARFHFFLCGFICYFVHSALASNSSSTLCFWFPLAHGNTSFELTINYTVCMPCPTSQAALQRLEPGRNMWCKIGHDRCEERDQDELLMSIPSGYDNLKLEGYYAWLAFLSFSYAAQFHPELFGIGNVSRVFVDKWHQFICAEHDGSNSTVSTGHNISALYAAYYHHQIDGGNWFHLEWLRPFFSSWLVLNISWFLRRSPVSPVSRRIYQILRPTRPQLPVSWSFRTSIVSDLMRSQQRKGKFPSGSRPNAVKPSALPNISR

SEQ ID NO: 45 - protein, 254 aa, Artificial Sequence
  AAE74526.1 PRRSV gp3
MANSCTFLYIFLCCSFLYSFCCAVVAGSNATYCFWFPLVRGNFSFELTVNYTVCPPCLTRQAATEAYEPGRSLWCRIGYDRCGEDDHDELGFVVPSGLSSEGHLTSVYAWLAFLSFSYTAQFHPEIFGIGNVSQVYVDIRHQFICAVHDGQNATLPRHDNISAVFQTYYQHQVDGGNWFHLEWLRPFFSSWLVLNVSWFLRRSPASHVSVRVLQTLRPTPPQRQALLSSKTSVALGIATRPLRRFAKSLSVVRR

SEQ ID NO: 46 - protein, 178 aa, Artificial Sequence
  AAE74537.1 PRRSV gp4
MASSLLFLMVGFKCLLVSQAFACKPCFSSSLADIKTNTTAAASFAVLQDIGCLRHRDSASEAIRKIPQCRTAIGTPVYITITANVTDENYLHSSDLLMLSSCLFYASEMSEKGFKVVFGNVSGIVAVCVNFTSYVQHVREFTQRSLVVDHVRLLHFMTPETMRWATVLACLFAILLAI

SEQ ID NO: 47 - protein, 178 aa, Artificial Sequence
  AAE74538.1 PRRSV gp4
MAASLLFLMVGFKCLLVSQAFACKPCFSSSLADIKTNTTAAASFAVLQDISCLRHRNSASEAIRKIPQCRTAIGTPMYITITANVTDENYLHSSDLLMLSSCLFYASEMSEKGFEVVFGNVSGIVAVCVNFTSYVQHVREFTQRSLMVDHVRLLHFMTPETMRWATVLACLFAILLAI

SEQ ID NO: 48 - protein, 178 aa, Artificial Sequence
  AAE74533.1 PRRSV gp4
MGASLLFLLVGFKCLLVSQAFACKPCFSSSLSDIKTNTTAAAGFAVLQDISCLRHRNSASEAIRKVPQCRTAIGTPVYITVTANVTDENYLHSSDLLMLSSCLFYASEMSEKGFKVVFGNVSGIVAVCVNFTSYVQHVKEFTQRSLVVDHVRLLHFMTPETMRWATVLACLFTILLAI

SEQ ID NO: 49 - protein, 183 aa, Artificial Sequence
  CAA01840.1 PRRSV gp4
MAAATLFFLAGAQHIMVSEAFACKPCFSTHLSDIETNTTAAAGFMVLQDINCFRPHGVSAAQEKISFGKSSQCREAVGTPQYITITANVTDESYLYNADLLMLSACLFYASEMSEKGFKVIFGNVSGVVSACVNFTDYVAHVTQHTQQHHLVIDHIRLLHFLTPSAMRWATTIACLFAILLAI

SEQ ID NO: 50 - protein, 183 aa, Artificial Sequence
  ABH73415.1 PRRSV gp4
MAAAILFLLAGAQHIMVSEAFACKPCFSTHLSDIKTNTTAAAGFMVLQDINCFRPHEVSATQREIPFRKSSQCREAVGTPQYITITANVTDESYLYNADLLMLSACLFYASEMSEKGFKVIFGNVSGVVSACVNFTDYVAHVTQHTQQHHLVIDHIRLLHFLTPSTMRWATTIACLFAILLAI

SEQ ID NO: 51 - protein, 178 aa, Artificial Sequence
  AAE68462.1 PRRSV gp4
MAASLLFLMVGFKCLLVSQAFACKPCFSSSLADIKTNTTAAASFAVLQDISCLRHRNSASEAIRKIPQCRTAIGTPVYITTTANVTDENYLHSSDLLMLSSCLFYASEMSEKGFKVVFGNVSGIVAVCVNFTSYVQHVREFTQRSLMVDHVRLLHFMTPETMRWATVLACLFAILLAI

SEQ ID NO: 52 - protein, 73 aa, Artificial Sequence
  AGX46781.1 PRRSV E
MGSMQSLFDKIGQLFVDAFTEFLVSIVDIIIFLAILFGFTIAGWLVVFCIRLVCSAILRTRPAIHPEQLQKIL

SEQ ID NO: 53 - protein, 73 aa, Artificial Sequence
  AED17147.1 PRRSV E
MGSIQSLFDKIGQLFVDAFTEFLVSIVDIIIFLAILFGFTIAGWLVVFCIRLVCSAVFRARPAIHPEQLQKIL

SEQ ID NO: 54 - protein, 73 aa, Artificial Sequence
  AED17148.1 PRRSV E
MGSIQSLFDKIGQLFVDAFTEFLVSIVDIIIFLAILFGFTIAGWLVVFCIRLVSSAVFRARPAIHPEQLQKIL

SEQ ID NO: 55 - protein, 69 aa, Artificial Sequence
  AGX46783.1 PRRSV E
MGSMQSLFDKIGQLFVDAFTEFLVSIVDIIIFLAILFGFTIAGWLVVFCIRLVCSALRRPAHEQLQKIL

SEQ ID NO: 56 - protein, 70 aa, Artificial Sequence
  AED17156.1 PRRSV E
MGSLWSKISQLFVDAFTEFLVSVVDIAIFLAILFGFTVAGWLLVFLLRVVCSALLRSRSAIHSPELSKVL

SEQ ID NO: 57 - protein, 73 aa, Artificial Sequence
  AIS76359.1 PRRSV E
MGSMQSLFDKIGQLFVDAFTEFLVSIVDIIIFLAILFGFTVAGWLVVFCIRLVFSAVLRARSTVHPEQLQKIL

SEQ ID NO: 58 - protein, 70 aa, Artificial Sequence
  ABU49670.1 PRRSV E
MGSLWSKISQLFVDAFTEFLVSVVDIVIFLAILFGFTVAGGLLVFFLRVVCSAILRSRSAIHSPELSKIL

SEQ ID NO: 59 - protein, 200 aa, Artificial Sequence
  VR2332 PRRSV gp5
MLEKCLTAGCCSRLLSLWCIVPFCFAVLANASNDSSSHLQLIYNLTLCELNGTDWLANKFDWAVESFVIFPVLTHIVSYGALTTSHFLDTVALVTVSTAGFVHGRYVLSSIYAVCALAALTCFVIRFAKNCMSWRYACTRYTNFLLDTKGRLYRWRSPVIIEKRGKVEVEGHLIDLKRVVLDGSVATPITRVSAEQWGRP

SEQ ID NO: 60 - protein, 201 aa, Artificial Sequence
  CAA01841.1 PRRSV gp5
MRCSHKLGRFLTPHSCFWWLFLLCTGLSWSFADGNGDSSTYQYIYNLTICELNGTDWLSSHFGWAVETFVLYPVATHILSLGFLTTSHFFDALGLGAVSTAGFVGGRYVLCSVYGACAFAAFVCFVIRAAKNCMACRYARTRFTNFIVDDRGRVHRWKSPIVVEKLGKAEVDGNLVTIKHVVLEGVKAQPLTRTSAEQWEA

SEQ ID NO: 61 - protein, 200 aa, Artificial Sequence
  ADA15222.1 PRRSV gp5
MLGKCLTAGCCSQLPFLWCIVPFCFAALVNASSSSSSQLQSIYNLTICELNGTDWLNKNFDWAVETFVIFPVLTHIVSYGALTTSHFLDAVGLITVSTAGYYHGRSVLSSVYAVCALAALICFVIRLTKNCMSWRYSCTRYTNFLLDSKGKLYRWRSPVIIEKGGKVEVDGHLIDLKRVVLDGSAATPVTKVSAEQWCRP

SEQ ID NO: 62 - protein, 46 aa, Artificial Sequence; identical to SEQ ID NO: 31
  AFS30909.1 PRRSV gp5a

SEQ ID NO: 63 - protein, 51 aa, Artificial Sequence
  AGK45334.1 PRRSV gp5a
MFKYVGELLDRGLLLAIAFFVVYRAVLFYCARQRQRKQQLLLPVDLQLDAM

SEQ ID NO: 64 - protein, 51 aa, Artificial Sequence
  AFU75332.1 PRRSV gp5a
MFKYVGEMLDRGLLLAIAFFVVYRAVLFHCARRRQRQQQLSSAIDLQLDAM

SEQ ID NO: 65 - protein, 46 aa, Artificial Sequence
  AGW23843.1 PRRSV gp5a
MFKYVGEMLDRGLLLTIAFFVVYRAVLVCCARQSRKRQQLPLTVDI

SEQ ID NO: 66 - protein, 152 aa, PRRSV VR2332
MDAMKRGLCCVLLLCGAVFVSPSDYKDDDDKGGSSNDSSSHLQLIYNLTLCELNGTDWLANKFDWAVESFVIFPVLTHIVSYGALTTSHFLDTVALVTVSTAGFVHGRYVLSSIYAVCALAALTCFVIRFAKLKHTKKRQIYTDIEMNRLGK

SEQ ID NO: 67 - DNA, 459 bp, PRRSV VR2332
atggatgctatgaaacggggactgtgctgcgtgctgctgctctgtggggctgtcttcgtgtcaccttctgattataaggacgatgacgataaaggaggaagtagcaatgacagctcctctcacctgcagctcatctacaacctgaccctctgcgagctgaatggaacagactggctcgctaacaagttcgattgggcagtggaatccttcgtcatctttcccgtgctgactcacattgtgagctatggggccctgaccacatcccatttcctggatacagtggccctcgtgactgtctctaccgctggctttgtccatggacgctacgtgctgtcaagtatctatgcagtctgcgccctggccgctctcacctgtttcgtgattagatttgcaaagctgaagcatacaaagaagcggcagatttacactgacattgagatgaatagactgggcaaatga

SEQ ID NO: 68 - protein, 155 aa, PRRSV VR2332
MDAMKRGLCCVLLLCGAVFVSPYPYDVPDYAGGSGSSLDDFCHDSTAPQKVLLAFSITYTPVMIYALKVSRGRLLGLLHLLIFLNCAFTFGYMTFAHFQSTNKVALTMGAVVALLWGVYSAIETWKFITSRCRLKLKHTKKRQIYTDIEMNRLGK

SEQ ID NO: 69 - DNA, 468 bp, PRRSV VR2332
atggatgctatgaaacggggactgtgctgcgtgctgctgctctgtggggctgtcttcgtgtcaccttacccctatgacgtgccagattacgcaggaggaagtgggtcaagcctcgacgatttttgtcacgattcaacagcacctcagaaagtcctcctcgccttcagcatcacatacactccagtcatgatctacgccctgaaggtgagtaggggcagactgctcggactgctccacctgctcattttcctgaactgcgcattcacttttggctatatgaccttcgcccattttcagtccaccaacaaggtggctctgacaatgggagcagtggtcgctctgctctggggggtctacagcgccatcgagacatggaagtttattacttcccgatgccgactgaagctgaagcatacaaagaagcggcagatttacactgacattgagatgaatagactgggcaaatga

SEQ ID NO: 70 - DNA, 747 bp, PRRSV
atgcaatggggtcactgtggagtaaaatcagccagctgttcgtggacgccttcactgagttccttgttagtgtggttgatattgccattttccttgccatactgtttgggttcaccgtcgcaggatggttactggtctttcttctcagagtggtttgctccgcgcttctccgttcgcgctctgccattcactctcccgaactatcgaaggtcctatgaaggcttgttgcccaactgcagaccggatgtcccacaatttgcagtcaagcacccattgggtatgttttggcacatgcgagtttcccacttgattgatgagatggtctctcgtcgcatttaccagaccatggaacattcaggtcaagcggcctggaagcaggtggttggtgaggccactctcacgaagctgtcagggctcgatatagttactcatttccaacacctggccgcagtggaggcggattcttgccgctttctcagctcacgactcgtgatgctaaaaaatcttgccgttggcaatgtgagcctacagtacaacaccacgttggaccgcgttgagctcatcttccccacgccaggtacgaggcccaagttgaccgatttcagacaatggctcatcagtgtgcacgcttccattttttcctctgtggcttcatctgttaccttgttcatagtgctttggcttcgaattccagctctacgctatgtttttggtttccattggcccacggcaacacatcattcgagc

SEQ ID NO: 71 - protein, 249 aa, PRRSV; identical to SEQ ID NO: 37

SEQ ID NO: 72 - DNA, 795 bp, PRRSV
atggctcatcagtgtgcacgcttccattttttcctctgtggcttcatctgttaccttgttcatagtgctttggcttcgaattccagctctacgctatgtttttggtttccattggcccacggcaacacatcattcgagctgaccatcaactacaccatatgcatgccctgttctaccagtcaagcggctcgccaaaggctcgagcccggtcgtaacatgtggtgcaaaatagggcatgacaggtgtgaggagcgtgaccatgatgagttgttaatgtccatcccgtccgggtacgacaacctcaaacttgagggttattatgcttggctggcttttttgtccttttcctacgcggcccaattccatccggagttgttcgggatagggaatgtgtcgcgcgtcttcgtggacaagcgacaccagttcatttgtgccgagcatgatggacacaattcaaccgtatctaccggacacaacatctccgcattatatgcggcatattaccaccaccaaatagacgggggcaattggttccatttggaatggctgcggccactcttttcttcctggctggtgctcaacatatcatggtttctgaggcgttcgcctgtaagccctgtttctcgacgcatctatcagatattgagaccaacacgaccgcggctgccggtttcatggtccttcaggacatcaattgtttccgacctcacggggtctcagcagcgcaagagaaaatttccttcggaaagtcgtcccaatgtcgtgaagccgtcggtactccccagtacatcacga

SEQ ID NO: 73 - protein, 158 aa, PRRSV
MAHQCARFHFFLCGFICYLVHSALASNSSSTLCFWFPLAHGNTSFELTINYTICMPCSTSQAARQRLEPGRNMWCKIGHDRCEERDHDELLMSIPSGYDNLKLEGYYAWLAFLSFSYAAQFHPELFGIGNVSRVFVDKRHQFICAEHDGHNSTVSTGH

SEQ ID NO: 74 - DNA, 549 bp, PRRSV
atggctgcggccactcttttcttcctggctggtgctcaacatatcatggtttctgaggcgttcgcctgtaagccctgtttctcgacgcatctatcagatattgagaccaacacgaccgcggctgccggtttcatggtccttcaggacatcaattgtttccgacctcacggggtctcagcagcgcaagagaaaatttccttcggaaagtcgtcccaatgtcgtgaagccgtcggtactccccagtacatcacgataacggctaacgtgaccgacgaatcatacttgtacaacgcggacctgctgatgctttctgcgtgccttttctacgcctcagaaatgagcgagaaaggcttcaaagtcatctttgggaatgtctctggcgttgtttctgcttgtgtcaatttcacagattatgtggcccatgtgacccaacatacccagcagcatcatctggtaattgatcacattcggttgctgcatttcctgacaccatctgcaatgaggtgggctacaaccattgcttgtttgttcgccattctcttggcaata

SEQ ID NO: 75 - protein, 183 aa, PRRSV; identical to SEQ ID NO: 49

SEQ ID NO: 76 - DNA, 603 bp, PRRSV
atgagatgttctcacaaattggggcgtttcttgactccgcactcttgcttctggtggctttttttgctgtgtaccggcttgtcctggtcctttgccgatggcaacggcgacagctcgacataccaatacatatataacttgacgatatgcgagctgaatgggaccgactggttgtccagccattttggttgggcagtcgagacctttgtgctttacccggttgccactcatatcctctcactgggttttctcacaacaagccatttttttgacgcgctcggtctcggcgctgtatccactgcaggatttgttggcgggcggtacgtactctgcagcgtctacggcgcttgtgctttcgcagcgttcgtatgttttgtcatccgtgctgctaaaaattgcatggcctgccgctatgcccgtacccggtttaccaacttcattgtggacgaccgggggagagttcatcgatggaagtctccaatagtggtagaaaaattgggcaaagccgaagtcgatggcaacctcgtcaccatcaaacatgtcgtcctcgaaggggttaaagctcaacccttgacgaggacttcggctgagcaatgggaggcc

SEQ ID NO: 77 - protein, 201 aa, PRRSV; identical to SEQ ID NO: 60

SEQ ID NO: 78 - DNA, 519 bp, PRRSV
atgggaggcctagacgatttttgcaacgatcctatcgccgcacaaaagctcgtgctagcctttagcatcacatacacacctataatgatatacgcccttaaggtgtcacgcggccgactcctggggctgttgcacatcctaatatttctgaactgttcctttacattcggatacatgacatatgtgcattttcaatccaccaaccgtgtcgcacttaccctgggggctgttgtcgcccttctgtggggtgtttacagcttcacagagtcatggaagtttatcacttccagatgcagattgtgttgccttggccggcgatacattctggcccctgcccatcacgtagaaagtgctgcaggtctccattcaatctcagcgtctggtaaccgagcatacgctgtgagaaagcccggactaacatcagtgaacggcactctagtaccaggacttcggagcctcgtgctgggcggcaaacgagctgttaaacgaggagtggttaacctcgtcaagtatggccgg

SEQ ID NO: 79 - protein, 173 aa, PRRSV
MGGLDDFCNDPIAAQKLVLAFSITYTPIMIYALKVSRGRLLGLLHILIFLNCSFTFGYMTYVHFQSTNRVALTLGAVVALLWGVYSFTESWKFITSRCRLCCLGRRYILAPAHHVESAAGLHSISASGNRAYAVRKPGLTSVNGTLVPGLRSLVLGGKRAVKRGVVNLVKYGR

SEQ ID NO: 80 - protein, 249 aa, Artificial Sequence
  Gp2 of PRRSV related to Lelystad PRRSV
MQWGHCGVKSASCSWTPSLSSLLVWLILSFSLPYCLGSPSQDGYWSFFSEWFAPRFSVRALPFTLPNYRRSYEGLLPNCRPDVPQFAVKHPLGMFWHMRVSHLIDEMVSRRIYQTMEHSGQAAWKQVVGEATLTKLSGLDIVTHFQHLAAVEADSCRFLSSRLVMLKNLAVGNVSLQYNTTLDRVELIFPTPGTRPKLTDFRQWLVSVHASIFSSVASSVTLFIVLWLRIPALRYVFGFHWPTATHHSS

SEQ ID NO: 81 - protein, 249 aa, Artificial Sequence
  Gp2 of PRRSV related to Lelystad PRRSV
MQWGHCGVKSASCSWTPSLSSLLVWLILSFSLPYCLGSPSQDGYWSFFSEWFAPRFSVRALPFTLPNYRRSYEGLLPNCRPDVPQFAFKHPLGMLWHMRVSHLIDEMVSRRIYQTMEHSGQAAWKQVVGEATLTKLSGLDIVTHFQHLAAVEADSCRFLSSRLVMLKNLAVGNVSLQYNTTLDRVELIFPTPGTRPKLTDFRQWLISVHASIFSSVASSVTLFIVLWLRIPALRYVFGFHWPTATHHSS

SEQ ID NO: 82 - protein, 249 aa, Artificial Sequence
  Gp2 of PRRSV related to Lelystad PRRSV
MQWGHCGVKSASCSWTPSLSSLLVWLILSFSLPYCLGSPSQDGYWSFFSEWFAPRFSVRALPFTLPNYRRSYEGLLPNCRPDVPQFAFKHPLGMFWHMRVSHLIDEMVSRRIYQTMEHSGQAAWKQVVGEATLTKLSGLDIVTHFQYLAAVEADSCRFLSSRLVMLKNLAVGNVSLQYNTTLDRVELIFPTPGTRPKLTDFRQWLVSVHASIFSSVASSVTLFIVLWLRIPALRYVFGFHWPTATHHSS

SEQ ID NO: 83 - protein, 249 aa, Artificial Sequence
  Gp2 of PRRSV related to Lelystad PRRSV
MQWGHCGVKSASCSWTPSLSSLLVWLILSFSLPYCLGSPSQDGYWSFFSEWFAPRFSVRALPFTLPNYRRSYEGLLPNCRPDVPQFAVKHPLGMFWHMRVSHLIDEMVSRRIYQTMEHSGQAAWKQVVGEATLTKLSGLDIVTHFQHLAAVEADSCRFLSSRLVMLKNLAVGNVSLQYNTTLDRVELIFPTPGTRPKLTDFRQWLISVHASIFSSVASSVTLFVVLWLRIPILRYVFGFHWPTATHHLS

SEQ ID NO: 84 - protein, 249 aa, Artificial Sequence
  Gp2 of PRRSV related to Lelystad PRRSV
MQWGHCGVRSASCSWTPSLSSLLVWLILSFFLPYCLGSPSQDGYWSFFSEWFAPRFSVRALPFTLPNYRRSYEGLLPNCRPDVPQFAVKHPLGMFWHMRVSHLIDEMVSRRIYQTMEHSGQAAWKHVVGEATLTKLSGLDIVTHFQHLAAVEADSCRFLSSRLVMLKNLAVGNVSLQYNTTLNRVELIFPTPGTRPKLTDFRQWLISVHASIFSSVASSVTLFTVLWLRIPALRYVFGFHWPTATHHSS

SEQ ID NO: 85 - protein, 249 aa, Artificial Sequence
  Gp2 of PRRSV related to Lelystad PRRSV
MQWGHCGVKSASCSWTPSLSSLLVWLTLSFSLPYCLGSPSQDGYWSFFSEWFAPRFSVRALPFTLPNYRRSYEGLLPNCRPDVPQFALKHPLGMLWHMRVSHLIDEMVSRRIYQTLEHSGQAAWKQAVGEATLTKLSRLDIVTHFQHLAAVEADSCRFLSSRLVMLKNLAVGNVSLQYNTTLDRVELIFPTPGTRPKLTDFRQWLISVHASIFSSVASSVTLFIVLWLRIPALRYVFGFHWPTATHHSS

SEQ ID NO: 86 - protein, 249 aa, Artificial Sequence
  Gp2 of PRRSV related to Lelystad PRRSV
MQWGHCGVKLASCSWTPSLSSLLVWLILSFSLPYCLGSPSQDGYWSFFSEWFAPRFSVRALPFTLPNYRRSYESLLPNCRPDVPQFAVKHPLGMLWHMRVSHLIDEMVSRRIYRTMEHSGQAAWKQVVSEATLTKLSGLDIVTHFQHLAAVEADSCRFLSSRLVMLKNLAVGNVSLQYNTTLDHVELIFPTPGTRPKLTDFRQWLISVHASIFSSVASSVTLFIVFWLRIPAVRYVFGFHWPTATHHSS

SEQ ID NO: 87 - protein, 249 aa, Artificial Sequence
  Gp2 of PRRSV related to Lelystad PRRSV
MQWGHCGVKLASCSWTLSLNSLLVWLILSFSLPYCLGSPSQDGYWSFFSEWFAPRFSVRALPFTLPNYRRSYEGLLPNCKPDVPQFAFKHPLGMFWHMRVSHLIDEMVSRRIYQTMEHSGQAAWKQVVGEATLTKLSRLDIVTHFQHLAAVEADSCRFLSSRLVMLKNLVVGNVSLQYNTTLDRVELVFPTPGARPKLTDFRQWLVSVHASIFSSVTSSVTLFIVLWLRIPALRYVFGFHWPTATHHSS

SEQ ID NO: 88 - protein, 249 aa, Artificial Sequence
  Gp2 of PRRSV related to Lelystad PRRSV
MQWGHCGVKLASCSWTPSLSSSLVWLILLSSLPYCLGSPSQDGYWSFFSEWFAPRFSVRALPFTLPNYRRSYESLLPNCRPDVPQFAFKHPLGILWHMRVSHLIDEMVSRRIYRTMEHSGQAAWKQVVSEATLTKLSGLDIVAHFQHLAAAEADSCRFLSSRLVMLKNLAVGNVSLQYNTTLDQVELIFPTPGTRPKLTDFRQWLISVHASIFSSVASSVTLFIVFWLRIPAVRYVFGFHWPTATRHSS

SEQ ID NO: 89 - protein, 249 aa, Artificial Sequence
  Gp2 of PRRSV related to Lelystad PRRSV
MQWGHYGAKSANCLWMPSLSSLLVWLISLFSLPYCLGSRSQGGYWSFFSGWFAPRFSVRALPFTLPNYRKSYEGLLPNCRPDVPSFAFKHPLGMFWHVRVSHLIDEMVSRRIYQTMEHSGQAAWKQVVSEATLTRLSDLDIVTHFQHLAAVEADSCRFLSSRLVMLKNLAVGNVSLQYNTTLDRVELIFPTPGTRPKLTDFRQWLVSVHASIFSSVASSVTLFIVLWLRIPTLRYVFGFHWPTATHHSS

SEQ ID NO: 90 - protein, 265 aa, Artificial Sequence
  Gp3 of PRRSV related to Lelystad PRRSV
MAHQCARFHFFLCGFICYLVHSALASNSSSTLCFWFPLAHGNTSFELTINYTICMPCSTSQAARQRLEPGRNMWCKIGHDRCEERDHDELLMSIPSGYDNLKLEGYYAWLAFLSFSYAAQFHPELFGIGNVSRVFVDKRHQFICAEHDGHNSTVSTGHNISALYAAYYHHQIDGGNWFHLEWLRPLFSSWLVLNISWFLRRSPVSPVSRRIYQILRPTRPRLPVSWSFRTSIVSDLTGSQQRKRKLPSESRPNVVKPSVLPSTSR

SEQ ID NO: 91 - protein, 265 aa, Artificial Sequence
  Gp3 of PRRSV related to Lelystad PRRSV
MAHQCARFHFFLCGFICYLVHSALASNSSYTLCFWFPLAHGNTSFELTINYTISMPCSTSQAARQRLEPGRNMWCKIGHDRCEERDHDELLMSIPSGYDNLKLEGYYAWLAFLSFSYAAQFHPELFGIGNVSRVFVDKRHQFICAEHDGQGSTVSTGHNISALYAAYYHHQIDGGNWFHLEWLRPLFSSWLVLNISWFLRRSPVSPVSRRIYHILRPTRPRLPVSWSFRTSIVSDLTGSQQRKRKFPSESRPNVVKPSVLPNTSR

SEQ ID NO: 92 - protein, 265 aa, Artificial Sequence
  Gp3 of PRRSV related to Lelystad PRRSV
MAHQCACFHFFLCGFICYLVHSALASNSSSTLCFWFPLAHGNTSFELTINYTICMPCLTSQAANQRLEPGRNMWCKIGHDRCEERDHDELLMSIPSGYDNLKLEGYYAWLAFLSFSYAAQFHPELFGIGNVSRVFVDKRHQFICAEHDGQNSTVSTGHNISASYAAYYHHQIDGGNWFHLEWLRPLFSSWLVLNISWFLRRSPVSPVSRRIYQILRPTRPRLPVSWSFRTSIVSDLTGSQQRKGKFPSENRPNVVKPSALPNTSR

SEQ ID NO: 93 - protein, 265 aa, Artificial Sequence
  Gp3 of PRRSV related to Lelystad PRRSV
MAHQCARFHFFLCGLIRYLVHSAVASNSSSTLCFWFPLAHGNTSFELTINYTICMPCSTSHAARQRLEPGRNMWCKIGHDRCEERDHDELLMPIPPGYDNLKLEGYYAWLAFLSFSYAAQFHPELFGIGNVSRVFVDKQHQFICAEHDGQNSTVSTGHNISALYAAYYHHQIDGGNWFHLEWLRPLFSSWLVLNISWFLRRSPVSPVSRRIYQILRQTRPRLPVSWSFRTSIVSDLTRSQQRKRKFPSESRPNVVKPSVLPSTSR

SEQ ID NO: 94 - protein, 265 aa, Artificial Sequence; identical to SEQ ID NO: 93
  Gp3 of PRRSV related to Lelystad PRRSV

SEQ ID NO: 95 - protein, 265 aa, Artificial Sequence
  Gp3 of PRRSV related to Lelystad PRRSV
  misc_feature (60)..(60): Xaa can be any naturally occurring amino acid
MAHQCARFHFFLCGFICYLVHSTLASNSSFTLCFWFPLAHGNTSFELTINYTICMPCSTXQAAHQRLEPGRNMWCKIGHDKCEERDHNELLMPIPPGYDNLKLEGYYAWLAFLSFSYAAQFHPELFGIGNVSRVFVDKRHQFICAEHDGLNSTVSTGHNISALYAAYYHHQIDGGNWFHLEWLRPLFSSWLVLNISWFLRRSPVSPVSRRIYQILRPTRPQLPVSWSFRTSIVSDLTRYQQRKRKFPSESRPNVVKPSVLPSTSR

SEQ ID NO: 96 - protein, 265 aa, Artificial Sequence; identical to SEQ ID NO: 44
  Gp3 of PRRSV related to Lelystad PRRSV

SEQ ID NO: 97 - protein, 261 aa, Artificial Sequence
  Gp3 of PRRSV related to Lelystad PRRSV
MAHQCARFHFFLCGFISYLVHSALASNSSSTLCFWFPLAHGNTSFELTINYTICMPCLTSQAAQQRLEPGRTMWCKIGHTTCEERDHDELSMTIPSGYDNLKLEGYYAWLAFLSFSYAAQFHPELFGIGNVSRVFVDKRHQFICAEHDGPNSTVSIGHNISALYAAYYHHQIDGGNWFHLEWLRPFFSSWLVLNISWFLRRSPVSPASRLIYQILRPTRPRLPVSWSFRTSIVPGLTGPQQRKRESRLNVVKPLVPPSTSR

SEQ ID NO: 98 - protein, 260 aa, Artificial Sequence
  Gp3 of PRRSV related to Lelystad PRRSV
MAHQCARFHLFLCGFICYSIHSALASDSNSTLCFWFPLAHGNTSFELTINYTICMPCLTSHAASQRLEPGRNMWCKIGHSRCEERDHDELLMSIPSGYDNLKLEGYYAWLAFLSFSYAAQFHPELFGIGNVSRVFVDKRHQFICAEHDGQNSTVSIGHNISALYAVYYHHQIDGGNWFHLEWLRPFFSSWLVLNISWFLRRSPASPVSRRIYQILKPTRPRLPVSWSFKTSVAAAQQRKMKVSGSRPNVAKPSAPLNTSR

SEQ ID NO: 99 - protein, 265 aa, Artificial Sequence
  Gp3 of PRRSV related to Lelystad PRRSV
MAHQCARLHFFLCGFVSYLVHSSLASNSSYTLCFWFPLAHGNTSFELTINYTICMPCTTSQAAQQRLEPGRNMWCRIGHTSCEERDHDELSMTIPSGYDNLKLEGYYAWLAFLSFSYTAQFHPELFGIGNVSRVFVDKRHQFICAEHDGQNSTVSITHNISALYAVYYHHQVDGGNWFHLEWLRPFFSSWLVLNISWFLRRSPASPVSRRIYQILRPTRPRLPVSWSFKTSPVPGLTGHQKGRKATFTTSHLNVVKPSAFPSTSR

SEQ ID NO: 100 - protein, 183 aa, Artificial Sequence
  Gp4 of PRRSV related to Lelystad PRRSV
MAAATLFLLAGAQHIMVSEAFACKPCFSTHLSDIETNTTAAAGFMVLQDINCFRPHGVSAAQEKISFGKSSQCREAVGTPQYITITANVTDESYLYNADLLMLSACLFYASEMSEKGFKVIFGNVSGVVSACVNFTDYVAHVTQHTQQHHLVIDHIRLLHFLTPSAMRWATTIASLFAILLAI

SEQ ID NO: 101 - protein, 183 aa, Artificial Sequence
  Gp4 of PRRSV related to Lelystad PRRSV
MAAAILFLLAGAQHIMVSEAFACKPCFSTHLSDIETNTTAAAGFMVLQDINCLRPHGVSAAQEKTSFGKSSQCREAVGTPQYITITANVTDESYLYNADLLMLSACLFYASEMSEKGFKVIFGNVSGVVSACVNFTDYVAHVTQHTQQHHLVIDHIRLLHFLTPSAMRWATTIACLFAILLAI

SEQ ID NO: 102 - protein, 183 aa, Artificial Sequence
  Gp4 of PRRSV related to Lelystad PRRSV
MAAATLFLLAGAQYIMVSEAFACKPCFSTHLSDIETNTTAAAGFMVLQDINCLRPHGVSAAQEEIPFGKSSQCREAVGTPQYITITANVTDESYLYNADLLMLSACLFHASEMSEKGFKVIFGNVSGVVSACVNFTDYVAHVTQHTQQHHLVIDHIRLLHFLTPSAMRWATTIACLFAILLAI

SEQ ID NO: 103 - protein, 183 aa, Artificial Sequence
  Gp4 of PRRSV related to Lelystad PRRSV
MAAATLFLLAGAQYIMVSEAFACKPCFSTHLSDIETNTTAAAGFMVLQDINCLRPHGVSAAQEEIPFGKSSQCREAVGTPQYITITANVTDESYLYNADLLMLSACLFHASEMSGKGFKVIFWNVSGVVSACVNFTDYVAHVTQHTQQHHLVIDHIRLLHFLTPSAMRWATTIACLFAILLAI

SEQ ID NO: 104 - protein, 183 aa, Artificial Sequence
  Gp4 of PRRSV related to Lelystad PRRSV
MAAATLFLLAGAQYIMVSEAFACKPCFSTHLSDIKTNTTAAAGFMVLQNINCLRPHGVPAAQEKIPLEKSSQCREAVGTPQYITITANVTDESYLYNADLLMLSACLFYASEMSEKGFKVIFGNVSGVVSACVNFTDYVAHVTQHTQQHHLVIDHIRLPHFLTPSAMRWATTIACLFAILLAI

SEQ ID NO: 105 - protein, 183 aa, Artificial Sequence
  Gp4 of PRRSV related to Lelystad PRRSV
MAAAILFLLAGAQHIMVSEAFACKPCFSTHLSDIKTNTTASAGFMVLQDINCFRLHGVPAAQKTNSFGKPSQCREAVGTPQYITITANVTDESYLYNADLLMLSACLFYASEMSEKGFKVIFGNVSGVVSACVNFTDYVAHVTQHTQQHHLVIDHIRLLHFLTPSAMRWATTIACLFAVLLAI

SEQ ID NO: 106 - protein, 183 aa, Artificial Sequence
  Gp4 of PRRSV related to Lelystad PRRSV
MAAAILFLLAGAQYLMVSEAFACKPCFSTHLSDIKTNTTAAAGFMVLQDINCLRPHGVSTAQENIPFGKPSQCREAVGIPQYITITANVTDESYLYNADLLMLSACLFYASEMSEKGFKVIFGNVSGVVSACVNFTDYVAHVIQHTQQHHLVIDHIRLLHFLTPSTMRWATTIACLFAILLAI

SEQ ID NO: 107 - protein, 183 aa, Artificial Sequence
  Gp4 of PRRSV related to Lelystad PRRSV
MATAILFLLASAQHLVVSEAFACKPCFSTHLSNIETNTTAAAGFLVLQDISCVQLRGGQQTSQSVTHGKPSQCREAIGTPQYITITANVTDESYLYNADLLMLSACLFYASEMSEKGFKVIFGNVSGVVSACINFTDYVAHVTQHTQQHHLIIDHVRLLHFLTPSAMRWVTTIACLFAILLAI

SEQ ID NO: 108 - protein, 183 aa, Artificial Sequence
  Gp4 of PRRSV related to Lelystad PRRSV
MAAAFLFLLVGAQYFMVSEAFACKPCFSTHLSDIETNTTAAAGFMVLQDISCLRPYGVSATHENISFGKPSQCREAVGIPQYITITANVTDESYLYNADLLMLSACLFYASEMSEKGFKVIFGNVSGVVSACVNFTDYVAHVIQHTQQHHLVIDHIRLLHFLTPSTMRWATTIACLFAILLAI

SEQ ID NO: 109 - protein, 183 aa, Artificial Sequence
  Gp4 of PRRSV related to Lelystad PRRSV
MATAVLFLLAGAQHLMVSEAFACKPCFSTHLSDIKTNTTAAAGFMVLQDINCLQPRGVSATHGSAPFKKSSQCREAVGTPQYITITANVTDESYLYNADLLMLSACLFYASEMSEKGFKVIFGNVSGVVSACVNFTDYVIHVTQHTQQHHLAIDHIRLLHFLTPSAMRWATTIACLFAILLAI

SEQ ID NO: 110 - protein, 200 aa, Artificial Sequence
  Gp5 of PRRSV related to Lelystad PRRSV
MRCSHKLGRFLTPHSCFWWLFLLCTGLSWSFADGNGNSSTYQYIYNLTICELNGTDWLSSHFGWAVETFVFYPVATHILSLGFLTTSHFFDALGLGAVSTAGFVGGRYVLCSVYGACAFAAFVCFVIRAAKNCMACRYARTRFTNFIVDDRGRVHRWKSPIVVEKLGRAEVDGNLVTIKHVVLEGVKAQPLTRTSAEQWE

SEQ ID NO: 111 - protein, 201 aa, Artificial Sequence
  Gp5 of PRRSV related to Lelystad PRRSV
MRCSHKLGRFLTPHSCFWWFFLLCTGLSWSFADGNGDSSTYQYIYNLTICELNGTDWLSSHFGWAVETFVLYPVATHILSLGFLTTSHFFDALGLGAVSAAGFVGGRYVLCSVYGACAFAAFVCFVIRAAKNCMACRYARTRFTNFIVDDRGRVHRWKSPIVVEKLGKAEVDGNLVTIKHVVLEGVKAQPLTRTSAEQWEA

SEQ ID NO: 112 - protein, 201 aa, Artificial Sequence
  Gp5 of PRRSV related to Lelystad PRRSV
MRCSHKLGRFLTPHSCFWWLFLLCTGLSWSFADGNGSSSTYQYIYNLTICELNGTDWLSSHFSWAVETFVLYPVVTHILSLGFLTTSHFFDALGLGAVSTAGFVGGRYVLCSVYGACAFAAFVCFVIRAAKNCMACRYARTRFTNFIVDDRGRVHRWKSPIVVEKLGKAEVDGNLITIKHVVLEGVKAQPLTRTSAEQWEA

SEQ ID NO: 113 - protein, 201 aa, Artificial Sequence
  Gp5 of PRRSV related to Lelystad PRRSV
MRCSHKLGRFLTPHSCFWWLFLLCTGLSWSFADGNGDSSTYQYIYNLTICELNGTDWLSSHFGWAVETFVLYPVATHILSLGFLTTSHLFDALGLGVVSTAGLVGGRYVLCSVYGACAFAAFVCFVIRAAKNCMACRYARTRFTNFIVDDRGRVHRWRSPIVVEKLGKAEVDGNLVTIKHVVLEGVKAQPLTRTSAEQWEA

SEQ ID NO: 114 - protein, 201 aa, Artificial Sequence
  Gp5 of PRRSV related to Lelystad PRRSV
MRCSHKLGRFLTPHSCFWWLFLLCTGLSWSFADGNGDSSTYQYIYNLTICELNGTDWLSSHFGWAVETFVLYPVATHILSLGFLTTSHLFDALGLGVVSTAGLVGGRYVLCSAYGACAFAAFVCFVIRAAKNCMACRYARTRFTNFIVDDRGRVHRWKSPIVVENLGKAEVDGNLVTIKHVVLEGVKAQPLTRTSAEQWEA

SEQ ID NO: 115 - protein, 201 aa, Artificial Sequence
  Gp5 of PRRSV related to Lelystad PRRSV
MRCSHKLGRFLTPHSCFWWLFLLCTGLSWSFADGNGDSSTYQYIYNLTICELNGTDWLSSHFGWAVETFVLYPVATHILSLGFLTTSHLFDALGLGVVSTAGLVSGRYVLCSVYGACAFAAFVCFVIRAAKNCMACRYARTRFTNFIVDDRGRVHRWKSPIVVENLGKAEVDGNLVTIKHVVLEGVKAQPLTRTSAEQWEA

SEQ ID NO: 116 - protein, 201 aa, Artificial Sequence
  Gp5 of PRRSV related to Lelystad PRRSV
MRCSHKLGRFLTPHSCFWWLFLLCTGLSWSFADGNGDSSTYQYIYNLTICELNGTDWLSSHFGWAVETFVLYPVATHILSLGFLTTSHLVDALGLGVVSTAGLVGGRYVLCSVYGACAFAAFVCFVIRAAKNCMACRYARTRFTNFIVDDRGRVHRWKSPIVVENLGKAEVDGNLVTIKHVVLEGVKAQPLTRTSAEQWEA

SEQ ID NO: 117 - protein, 201 aa, Artificial Sequence
  Gp5 of PRRSV related to Lelystad PRRSV
MRCPHKLGRFLTPHSCFWWLFLLCTGLSWSFADGNGDSSTYQYIYNLTICELNGTDWLSSHLGWAVETFVLYPVATHILSLGFLTTSHLFDALGLGVVSTAGLIGGRYVLCSVYGACAFAAFVCFVIRAAKNCMACRYARTRFTNFIVDDRGRVHRWKSPIVVENLGKAEVDGNLVTIKHVVLEGVKAQPLTRTSAEQWEA

SEQ ID NO: 118 - protein, 201 aa, Artificial Sequence
  Gp5 of PRRSV related to Lelystad PRRSV
MRCSHKLGRFLTPHSCFWWLFLLCIGLSWSFADGNGSSSTYQYIYDLTICELNGTDWLSSHFGWAVETFVLYPVATHILSLGFLTTSHFFDALGLGAVSTAGFVGGRYVFCSVYGACAFAAFVCFVIRAAKNCMACRYARTRFTNFIVDDRGRVHRWKSPIVVEKLGKAEVDGNLVTIKHVVLEGYKAQPLTRTSAQQWEA

SEQ ID NO: 119 - protein, 201 aa, Artificial Sequence
  Gp5 of PRRSV related to Lelystad PRRSV
MSSSHKLGRFLTPHSCFWWLFLLCTGLSWSFADGNGNSSTYQYIYNLTICELNGTDWLSSHFGWAVETFVLYPVATHILSLGFLTTSHFFDALGLGAVSTAGFVGGRYVLCSVYGACAFAAFVCFVIRAAKNCMACRYARTRFTNFIVDDRGRVHRWKSPIVVEKLGKAEVGGNLVTIKHVVLEGVKAQPLTRTSAEQWRA

SEQ ID NO: 120 - protein, 173 aa, Artificial Sequence
  M of PRRSV related to Lelystad PRRSV
MGGLDDFCNDPIAAQKLVLAFSITYTPIMIYALKVSRGRLLGLLHILIFLNCSFTFGYMTYVHFQSTNRVAFTLGAVVALLWGVYSFTESWKFITSRCRLCCLGRRYILAPAHHVESAAGLHSISASGNRAYAVRKPGLTSVNGTLVPGLRSLVLGGKRAVKRGVVNLVKYGR

SEQ ID NO: 121 - protein, 173 aa, Artificial Sequence
  M of PRRSV related to Lelystad PRRSV
MGSLDDFCYDSIAAQKLVLAFSITYTPIMIYALKVSRGRLLGLLHILIFLNCSFTFGYMTYVHFQSTNRVALTLGAAVALLWGVYSFTESWKFITSRCRLCCLGRRYILAPAHHVESAAGLHPISASGNRAYAVRKPGLTSVNGTLVPGLRNLVLGGKRAVKRGVVNLVKYGR

SEQ ID NO: 122 - protein, 173 aa, Artificial Sequence
  M of PRRSV related to Lelystad PRRSV
MGSLDDFCNDSAAVQKLVLAFSITYTPIMIYALKVSRGRLLGLLHILIFLNCSFTFGYMTHVHFQSTNRVAFTLGAVVALLWGVYSFTESWKFITSRCRLCCLGRRYILAPAHHVESAAGLHSIPASGNRAYAVRKPGLTSVNGTLVPGLRSLVLGGKRAVKRGVVNLVKYGR

SEQ ID NO: 123 - protein, 173 aa, Artificial Sequence
  M of PRRSV related to Lelystad PRRSV
MGSLDRFCNEPDAVQQLVLAFSITYTPIMIYALKVSRGRLLGLLHILIFLNCSFTFGYMTYVHFQSTNRVALTLGAVVTLLWGVYSFTESWKFITSRCRLCCLGRRYILAPAHHVESAAGLHSIPASGNRAYAVRKPGLTSVNGTLVPGLRGLVLGGKRAVKRGVVNLVKYGR

SEQ ID NO: 124 - protein, 173 aa, Artificial Sequence
  M of PRRSV related to Lelystad PRRSV
MGSLDGFCDEPAAVQKLVLAFSTTYTPIMIYALKVSRGRLLGLLHILIFLNCSFTFGYMTYVHFQSINRVAFTLGAVVALLWGVYSFTESWKSITSRCRLCCLGRRYILAPAHHVESAAGLHSIPASGNRAYAVRKPGLTSVNGTLVPGLRSLVLGGKRAVKRGVVNLVKYGR

SEQ ID NO: 125 - protein, 173 aa, Artificial Sequence
  M of PRRSV related to Lelystad PRRSV
MGSIDGFCDDPAAVQKLVLAFSITYTPIMIYALKVSRGRLLGLLHILIFLNCSFAFGYMTYVHFQSTNRVAITLGAVVALLWGVYSFIESWKFITFRCRLCCLGRRYILAPAHHVESAAGLHPIPASGNRAYAVRKPGLTSVNGTLVPGLRSLVLGGKRAVKRGVVNLVKYGR

SEQ ID NO: 126 - protein, 173 aa, Artificial Sequence
  M of PRRSV related to Lelystad PRRSV
MGGLDDFCFDHYSAQKLVLAFSITYTPIMIYALKASRGRLLGLLHILIFLNCAFTFGYMTYVHFQSTHRVALTMGAVVALLWGVYSFIESWKFITSRCRLCCLGRRYILAPAHHVESAAGLHPIPASGNRGYALRKPGLTSVNGTLVPGLRSLVLGGKRAVRRGVVNLVKYGR

SEQ ID NO: 127 - protein, 173 aa, Artificial Sequence
  M of PRRSV related to Lelystad PRRSV
MGGLDNFCYDSTAAQKVLLAFSITYTPIMIYALKVSRGRLLGLLHILIFLNCSFTFGYMTYEHFESTNRVALTMGAVVALLWGVYSFIESWKFVTFRCRLCCLGRQYILAPAHHVESAAGLHSIPASGNQAYAVRKPGLTSVNGTLVPGLRSLVLGGKRAVKRGLVNLVKYGR

SEQ ID NO: 128 - protein, 173 aa, Artificial Sequence
  M of PRRSV related to Lelystad PRRSV
MAGLDDFCYDSTAVQKLVLAFSITYTPIMIYALKVSRGRLLGLLHILIFLNCSFTFGYMTYVHFESSNRVAFTMGAVVTLLWGIYSFIESWKFVTSRCRLCCLGRRYILAPAHHVESAAGLHPIPASGNQAYAVRKPGLTSVNGTLVPGLRGLVLGGKRAVKRGMVNLVKYGR

SEQ ID NO: 129 - protein, 173 aa, Artificial Sequence
  M of PRRSV related to Lelystad PRRSV
MGSLDNFCHDPTAVQKVLLAFSITYTPVMIYALKVSRGRLLGLLHILIFLNCSFTFGYLTYVHFDSTNRVALTMGAVVALLWGIYSFIESWKFVVSRCRLCCLGRQYILAPAHHVESAAGLHPLPACGNQAFAVRKPGLTSVNGTLVPGLRSLVLGGKRAVKRGVVNLVKYGR

SEQ ID NO: 130 - protein, 70 aa, Artificial Sequence; identical to SEQ ID NO: 56
  E of PRRSV related to Lelystad PRRSV

SEQ ID NO: 131 - protein, 70 aa, Artificial Sequence
  E of PRRSV related to Lelystad PRRSV
MGSLWSKISQLFVDAFTEFLVSVVDIVIFLAILFGFTVAGWLLVFLLRVVCSALLRSRSAIHSPELSKVL

SEQ ID NO: 132 - protein, 70 aa, Artificial Sequence
  E of PRRSV related to Lelystad PRRSV
MGSLWSKISQLFVDAFTEFLVSVVDIVIFLAILFGFTVAGWLLVFLLRVVCSALLRSRSAVHSPELSKVL

SEQ ID NO: 133 - protein, 70 aa, Artificial Sequence
  E of PRRSV related to Lelystad PRRSV
MGSLWSKISQLFVDAFTEFLVSVVDIVIFLAILFGFTVAGWLLVFLLRVVCSAILRSRSAIHSPELSKVL

SEQ ID NO: 134 - protein, 70 aa, Artificial Sequence
  E of PRRSV related to Lelystad PRRSV
MGSLWSKISQLFVDAFTEFLVSVVDIVIFLAILFGFTVAGWLLVFLLRVVCSAFLRSRSAIHSPELSKVL

SEQ ID NO: 135 - protein, 70 aa, Artificial Sequence
  E of PRRSV related to Lelystad PRRSV
MGSLWSKITQLFVDAFTEFLVSVVDIIIFLAILFGFTVAGWLLVFLLRVVCSAILRSRSAIHSPELSKVL

SEQ ID NO: 136 - protein, 70 aa, Artificial Sequence
  E of PRRSV related to Lelystad PRRSV
MGSLWSKISQLFVDAFTEFLVSVVDIVIFLAILFGFTVAGWLLVFLLRLVCSAILRSRSAIHSPELSKVL

SEQ ID NO: 137 - protein, 70 aa, Artificial Sequence
  E of PRRSV related to Lelystad PRRSV
MGSLWSKISQLFVDAFTEFLVSVVDIVIFLAILFGFTVAGWLLVFLLRVVCSALLRSRSAIHPPELSKIL

SEQ ID NO: 138 - protein, 70 aa, Artificial Sequence
  E of PRRSV related to Lelystad PRRSV
MGSLWSKISQLFVDAFTEFLVSVVDIVIFLAILFGFTVAGWLLVFLFRLVCSAILRSRSAIHSSELSKVL

SEQ ID NO: 139 - protein, 70 aa, Artificial Sequence
  E of PRRSV related to Lelystad PRRSV
MGSLWSKISQLFVDAFTEFLVSVVDIVIFLAILFGFTVAGWLLVFLLRVVCSAFLRSRSAIHSSELSKVL